European Patent Specification EP 3 805 391 B1, published June 19, 2024. Title: Use of Yr4DS Gene of Aegilops Tauschii In Stripe Rust Resistance Breeding of Triticeae Plants. Applicant: SHANDONG AGRICULTURAL UNIVERSITY SICHUAN AGRICULTURAL UNIVERSITY. Application EP19811581.8. The sequence listing filed with the application follows.

SEQUENCE LISTING (63 sequences)

SEQ ID NO: 1 - DNA, 4266 bp, Aegilops tauschii'PI511383'
gcagctccacctaccgcagctggccggtcgtcggtccttgcatcgcatccaaggcgacgccggctccaccactgccgccaccactgattggtaccttaagctcccgtgaagctacaagggaggaggccccctcgcctcccatccattgttcctcaacagcttgggtgccgagctcccccaccaccacactagacgcgctgggattcattggatccgctccagcgagcgagccggattcagttcaccgagattatattcacccttcccgtctgccaactgattacctcccttttcccattctaccctgggtgaccactctgctcactctcactctttctttctcctctacgccggccgtgcacagcgcgacgccgacgaccgcatccccccgacgttgccgcagccgccatacaagtagaaggaccgagatggcaacctctcccagctttgtgctacaccgcaagtactaggagcattgctgaatgccggatatagatccccagatctaggccaagggtctcgctttctgctcactgttacttctatcatctctccaatcgatccaagttccagctcaagccactggaccctgcaactacttgcgagacagcacgggatatctatctctgcaacaagatccgtctctcatctctctagtcgattcaagtactagttcaagcgtgagcaaaccctgcaaccaatggcgggggttctggatgctttggcatcctacgtgaccaacatgctcaccgagatggctaaagaggaggtggccatgctaatcggcgtgtctgacgggatcaaagacctaagcatcaagcttggggacctcaagaatttccttgctgatgctgataggaggaacattaccgatgatagtgtgcgggggtgggtgggcgaactgaagcgtgccatgtacttggccactgacatcgtcgacctatgtcagctcaaggccatggagcaaggtcaaacaaaggacagggcgtgccggtgccttaaccctctgctcttttgcatgcggaatcccctccacgcccacgacatcggcacccgcatcaagctgctcaaccaaaatttggatgatatttgcaagaggggcagcagtttcaatttcatcaagctagaagcctaccaagaccaaaagaccactcggtctcccgccactgaccggaaaacaaattcactgattgagcggtccggtgtggttggagagaagatcgaggaggacacgagggcacttgtggaggtgcttacaagggaggcggtaggtgacaagagtggtcgcctcattgtggtcgccattgttggtatcggagggattggtaagactaccctcggcaagaaggtcttcaatgatgaggccatcgaaggcaagtttactaagaagatatggcttagcatcacacaagatttcaccgatgttgagttgttaagtacgaccatcactgccattggggcagatcttcctggagggggtggggctccagacaaggccctacttgtcgatgctctcaagaacgccatcaaggacaagaagttctttcttgtactagatgacctgtgggatgtcgatgcatggaacaaacatctaatgactccctttagctatggtggccccggtagtagagtcctcatcaccaccagacatgacactgtagcccgaagcatgaaagcctttcatccctaccatcatgttgacaaattagctccacaagatgcttggtcgttgctcaagaagcaggtagtcacaggagaggaaaatgaaccagaagttgatatgctagaagatattgggctgcagattatagcaaaatgtgatggcttaccacttgctgtaaaagttatgggtggactcctatgcaagaaggagaaaacacgacgtgattggcaagacgtcttgaatgatgatatgtggtcagtatctcaaatgtcaaaggaactaaattatgccatatatcttagctatgaggatttgtccccttacttaaaacagtgcttcttgcacttctccctcaaaccaaaaaagacagtgataactgatactgaaatggtgtccatgtgggttggtgaaggattggttgaaggagacacatatactcgtagtttggaagaagggaataagtactataaggagctaatagtaaggaaccttatagaggtagatacaaagtaccctagtcaacttatttgcaacatgcatgatgttattcgctcatttgctcaatttgtggctagggatgaaacactagtaggtcacaatggagatactatcaaaacaaatcttagatcaccgaattatcttagattatccatagaaacgaaaggagtgggatccgatgaatttgagtggagatatttaagagagcaaaaattgcttaggtctctaatattaactggaaacctcaaaagtcagcctggggattcgttgactatcttcccaagtctacgtcttttgcatatagaatcagcaaatattgctgcactagttgaatctatgtaccaactcaagcatttgagatatttggcattaaagaggactgatatgtgtagactaccagagaacatccatgagatgaaattcctacagcatattagccttgaaggttgtgaaagtttcatgaaacttcctgatagtattatcaagctgcaagggttgagatatcttgatatgggtgacacacgtgtaagtagtattcctaggggtttccgagctcttacaaatttgacttcactatttgggtttccagcctatattgatggtgactggtgtagtctggaagagttggggtctctttcccagctcaatgaactttcactacagagcctagaaaatgtatctagtgccttgttggctgaaaaggcaagggtaaatgcaaagaaacaacttaccgtacttgctttaaaatgtggtggtagagtgggacatgggttggtccaaggagaggtctctgagtctaaggaggaggagcaaataattgaggcggtgtttgatgtgctctgtcctcagccttgcatagaacacatcagaatagaaagatattttggtcgtcggctcccaggatggatggcgtccacagctatggtgcccctcgagagcttgaagattctatgcctcgaacacctgccctgctgcacccaactcccagatggcttgtgcaggctcccgtatttggagtggataaaagtgatgaatgctccagtaatcaagtgtattggtcctgaattcgttcaacagtacaatcagctgcaccgtccttcatctcagttggctgctacgtttcccaaactccagatgttggaatttcacggaatggaggaatgggaggagtgggtttgggagacggaagtgaaagctatgcccttattggaggaacttcgtatcacttcttgcagactgagccgtatgcctccaggacttatgtctcatgcaatggctttgaagaagctaacaatatggagcgtccaatgtctccactctctagagaactttgtttctgtagttgaactcgaattgggaaacatacctgaactggccatgatctccaatcttccaaaattacaaaaacttacaatcgagtgctgcccaaagctcgagatgctgcaggagatggctgcactccggagactcgagctgaccattttcaacagcgaaaatcaacttccggtctacctgcagactgtgaagcctagtaatttgctgctgacctgcaacctagcggtactcacttccatggctgagggtgaatctagctccgagtgggacaagttcagtcatatcaaccacgttgaggcttatgcagaggatggagaagatgagaagaaatggcacgtgttctacacatctgaatcctgcaacatagagacaaatattcatcaggatcgattggtcgaagaagaggagtaggctgaaactccagccgaacgaggaaggaccatatgatgcaaggatatataagtatgtctgctgttacaacttcaactagttttgagatcgaatccatgaagggatacggggaaaagcatcagccataatgccatatacacttacctgcagagattcacacatcatactaatttcttgtgaagtgtgacatatacagttacgaatttagagatgtaaacttcgtggcggactatccagctggtgaagaaacatggtgaccttggcaaggctctcctttgtttagtgcaagcaactaatggagtttagactactctgctttgctctgctctctgaaagcagctcaggttgcaggtcctctg

SEQ ID NO: 2 - protein, 1068 aa, Aegilops tauschii'PI511383'
MAGVLDALASYVTNMLTEMAKEEVAMLIGVSDGIKDLSIKLGDLKNFLADADRRNITDDSVRGWVGELKRAMYLATDIVDLCQLKAMEQGQTKDRACRCLNPLLFCMRNPLHAHDIGTRIKLLNQNLDDICKRGSSFNFIKLEAYQDQKTTRSPATDRKTNSLIERSGVVGEKIEEDTRALVEVLTREAVGDKSGRLIVVAIVGIGGIGKTTLGKKVFNDEAIEGKFTKKIWLSITQDFTDVELLSTTITAIGADLPGGGGAPDKALLVDALKNAIKDKKFFLVLDDLWDVDAWNKHLMTPFSYGGPGSRVLITTRHDTVARSMKAFHPYHHVDKLAPQDAWSLLKKQVVTGEENEPEVDMLEDIGLQIIAKCDGLPLAVKVMGGLLCKKEKTRRDWQDVLNDDMWSVSQMSKELNYAIYLSYEDLSPYLKQCFLHFSLKPKKTVITDTEMVSMWVGEGLVEGDTYTRSLEEGNKYYKELIVRNLIEVDTKYPSQLICNMHDVIRSFAQFVARDETLVGHNGDTIKTNLRSPNYLRLSIETKGVGSDEFEWRYLREQKLLRSLILTGNLKSQPGDSLTIFPSLRLLHIESANIAALVESMYQLKHLRYLALKRTDMCRLPENIHEMKFLQHISLEGCESFMKLPDSIIKLQGLRYLDMGDTRVSSIPRGFRALTNLTSLFGFPAYIDGDWCSLEELGSLSQLNELSLQSLENVSSALLAEKARVNAKKQLTVLALKCGGRVGHGLVQGEVSESKEEEQIIEAVFDVLCPQPCIEHIRIERYFGRRLPGWMASTAMVPLESLKILCLEHLPCCTQLPDGLCRLPYLEWIKVMNAPVIKCIGPEFVQQYNQLHRPSSQLAATFPKLQMLEFHGMEEWEEWVWETEVKAMPLLEELRITSCRLSRMPPGLMSHAMALKKLTIWSVQCLHSLENFVSVVELELGNIPELAMISNLPKLQKLTIECCPKLEMLQEMAALRRLELTIFNSENQLPVYLQTVKPSNLLLTCNLAVLTSMAEGESSSEWDKFSHINHVEAYAEDGEDEKKWHVFYTSESCNIETNIHQDRLVEEEE

SEQ ID NO: 3 - DNA, 3477 bp, Aegilops tauschii'PI511383'
gcagctccacctaccgcagctggccggtcgtcggtccttgcatcgcatccaaggcgacgccggctccaccactgccgccaccactgattggtaccttaagctcccgtgaagctacaagggaggaggccccctcgcctcccatccattgttcctcaacagcttgggtgccgagctcccccaccaccacactagacgcgctgggattcattggatccgctccagcgagcgagccggattcagttcaccgagattatattcacccttcccgtctgccaactgattacctcccttttcccattctaccctgggtgaccactctgctcactctcactctttctttctcctctacgccggccgtgcacagcgcgacgccgacgaccgcatccccccgacgttgccgcagccgccatacaagtagaaggaccgagatggcaacctctcccagctttgtgctacaccgcaagtactaggagcattgctgaatgccggatatagatccccagatctaggccaagggtctcgctttctgctcactgttacttctatcatctctccaatcgatccaagttccagctcaagccactggaccctgcaactacttgcgagacagcacgggatatctatctctgcaacaagatccgtctctcatctctctagtcgattcaagtactagttcaagcgtgagcaaaccctgcaaccaatggcgggggttctggatgctttggcatcctacgtgaccaacatgctcaccgagatggctaaagaggaggtggccatgctaatcggcgtgtctgacgggatcaaagacctaagcatcaagcttggggacctcaagaatttccttgctgatgctgataggaggaacattaccgatgatagtgtgcgggggtgggtgggcgaactgaagcgtgccatgtacttggccactgacatcgtcgacctatgtcagctcaaggccatggagcaaggtcaaacaaaggacagggcgtgccggtgccttaaccctctgctcttttgcatgcggaatcccctccacgcccacgacatcggcacccgcatcaagctgctcaaccaaaatttggatgatatttgcaagaggggcagcagtttcaatttcatcaagctagaagcctaccaagaccaaaagaccactcggtctcccgccactgaccggaaaacaaattcactgattgagcggtccggtgtggttggagagaagatcgaggaggacacgagggcacttgtggaggtgcttacaagggaggcggtaggtgacaagagtggtcgcctcattgtggtcgccattgttggtatcggagggattggtaagactaccctcggcaagaaggtcttcaatgatgaggccatcgaaggcaagtttactaagaagatatggcttagcatcacacaagatttcaccgatgttgagttgttaagtacgaccatcactgccattggggcagatcttcctggagggggtggggctccagacaaggccctacttgtcgatgctctcaagaacgccatcaaggacaagaagttctttcttgtactagatgacctgtgggatgtcgatgcatggaacaaacatctaatgactccctttagctatggtggccccggtagtagagtcctcatcaccaccagacatgacactgtagcccgaagcatgaaagcctttcatccctaccatcatgttgacaaattagctccacaagatgcttggtcgttgctcaagaagcaggtagtcacaggagaggaaaatgaaccagaagttgatatgctagaagatattgggctgcagattatagcaaaatgtgatggcttaccacttgctgtaaaagttatgggtggactcctatgcaagaaggagaaaacacgacgtgattggcaagacgtcttgaatgatgatatgtgcctatattgatggtgactggtgtagtctggaagagttggggtctctttcccagctcaatgaactttcactacagagcctagaaaatgtatctagtgccttgttggctgaaaaggcaagggtaaatgcaaagaaacaacttaccgtacttgctttaaaatgtggtggtagagtgggacatgggttggtccaaggagaggtctctgagtctaaggaggaggagcaaataattgaggcggtgtttgatgtgctctgtcctcagccttgcatagaacacatcagaatagaaagatattttggtcgtcggctcccaggatggatggcgtccacagctatggtgcccctcgagagcttgaagattctatgcctcgaacacctgccctgctgcacccaactcccagatggcttgtgcaggctcccgtatttggagtggataaaagtgatgaatgctccagtaatcaagtgtattggtcctgaattcgttcaacagtacaatcagctgcaccgtccttcatctcagttggctgctacgtttcccaaactccagatgttggaatttcacggaatggaggaatgggaggagtgggtttgggagacggaagtgaaagctatgcccttattggaggaacttcgtatcacttcttgcagactgagccgtatgcctccaggacttatgtctcatgcaatggctttgaagaagctaacaatatggagcgtccaatgtctccactctctagagaactttgtttctgtagttgaactcgaattgggaaacatacctgaactggccatgatctccaatcttccaaaattacaaaaacttacaatcgagtgctgcccaaagctcgagatgctgcaggagatggctgcactccggagactcgagctgaccattttcaacagcgaaaatcaacttccggtctacctgcagactgtgaagcctagtaatttgctgctgacctgcaacctagcggtactcacttccatggctgagggtgaatctagctccgagtgggacaagttcagtcatatcaaccacgttgaggcttatgcagaggatggagaagatgagaagaaatggcacgtgttctacacatctgaatcctgcaacatagagacaaatattcatcaggatcgattggtcgaagaagaggagtaggctgaaactccagccgaacgaggaaggaccatatgatgcaaggatatataaagattcacacatcatactaatttcttgtgaagtgtgacatatacagttacgaatttagagatgtaaacttcgtggcggactatccagctggtgaagaaacatggtgaccttggcaaggctctcctttgtttagtgcaagcaactaatggagtttagactactctgctttgctctgctctctgaaagcagctcaggttgcaggtcctctgaagcagctgcgtttttctttttcttttttcgcgggtgtctttcattcgttctctggaaaactatgtttatttctgatagatcaatcaatagtatactggaacactaaatactgttagaacaaacccaatcaaaatgtactaat

SEQ ID NO: 4 - protein, 408 aa, Aegilops tauschii'PI511383'
MAGVLDALASYVTNMLTEMAKEEVAMLIGVSDGIKDLSIKLGDLKNFLADADRRNITDDSVRGWVGELKRAMYLATDIVDLCQLKAMEQGQTKDRACRCLNPLLFCMRNPLHAHDIGTRIKLLNQNLDDICKRGSSFNFIKLEAYQDQKTTRSPATDRKTNSLIERSGVVGEKIEEDTRALVEVLTREAVGDKSGRLIVVAIVGIGGIGKTTLGKKVFNDEAIEGKFTKKIWLSITQDFTDVELLSTTITAIGADLPGGGGAPDKALLVDALKNAIKDKKFFLVLDDLWDVDAWNKHLMTPFSYGGPGSRVLITTRHDTVARSMKAFHPYHHVDKLAPQDAWSLLKKQVVTGEENEPEVDMLEDIGLQIIAKCDGLPLAVKVMGGLLCKKEKTRRDWQDVLNDDMCLY

SEQ ID NO: 5 - DNA, 2853 bp, Aegilops tauschii'PI511383'
gcagctccacctaccgcagctggccggtcgtcggtccttgcatcgcatccaaggcgacgccggctccaccactgccgccaccactgattggtaccttaagctcccgtgaagctacaagggaggaggccccctcgcctcccatccattgttcctcaacagcttgggtgccgagctcccccaccaccacactagacgcgctgggattcattggatccgctccagcgagcgagccggattcagttcaccgagattatattcacccttcccgtctgccaactgattacctcccttttcccattctaccctgggtgaccactctgctcactctcactctttctttctcctctacgccggccgtgcacagcgcgacgccgacgaccgcatccccccgacgttgccgcagccgccatacaagtagaaggaccgagatggcaacctctcccagctttgtgctacaccgcaagtactaggagcattgctgaatgccggatatagatccccagatctaggccaagggtctcgctttctgctcactgttacttctatcatctctccaatcgatccaagttccagctcaagccactggaccctgcaactacttgcgagacagcacgggatatctatctctgcaacaagatccgtctctcatctctctagtcgattcaagtactagttcaagcgtgagcaaaccctgcaaccaatggcgggggttctggatgctttggcatcctacgtgaccaacatgctcaccgagatggctaaagaggaggtggccatgctaatcggcgtgtctgacgggatcaaagacctaagcatcaagcttggggacctcaagaatttccttgctgatgctgataggaggaacattaccgatgatagtgtgcgggggtgggtgggcgaactgaagcgtgccatgtacttggccactgacatcgtcgacctatgtcagctcaaggccatggagcaaggtcaaacaaaggacagggcgtgccggtgccttaaccctctgctcttttgcatgcggaatcccctccacgcccacgacatcggcacccgcatcaagctgctcaaccaaaatttggatgatatttgcaagaggggcagcagtttcaatttcatcaagctagaagcctaccaagaccaaaagaccactcggtctcccgccactgaccggaaaacaaattcactgattgagcggtccggtgtggttggagagaagatcgaggaggacacgagggcacttgtggaggtgcttacaagggaggcggtaggtgacaagagtggtcgcctcattgtggtcgccattgttggtatcggagggattggtaagactaccctcggcaagaaggtcttcaatgatgaggccatcgaaggcaagtttactaagaagatatggcttagcatcacacaagatttcaccgatgttgagttgttaagtacgaccatcactgccattggggcagatcttcctggagggggtggggctccagacaaggccctacttgtcgatgctctcaagaacgccatcaaggacaagaagttctttcttgtactagatgacctgtgggatgtcgatgcatggaacaaacatctaatgactccctttagctatggtggccccggtagtagagtcctcatcaccaccagacatgacactgtagcccgaagcatgaaagcctttcatccctaccatcatgttgacaaattagctccacaagatgcttggtcgttgctcaagaagcaggtagtcacaggagaggaaaatgaaccagaagttgatatgctagaagatattgggctgcagattatagcaaaatgtgatggcttaccacttgctgtaaaagttatgggtggactcctatgcaagaaggagaaaacacgacgtgattggcaagacgtcttgaatgatgatatgtggtcagtatctcaaatgtcaaaggaactaaattatgccatatatcttagctatgaggatttgtccccttacttaaaacagtgcttcttgcacttctccctcaaaccaaaaaagacagtgataactgatactgaaatggtgtccatgtgggttggtgaaggattggttgaaggagacacatatactcgtagtttggaagaagggaataagtactataaggagctaatagtaaggaaccttatagaggatcgattggtggaagaagaggactagaccgaaactcctacggaacgagtttaggcgaaaggaccatatgatgcaaggatatacggatacctggaaagcatcagccataatgccatatacacttaacctgcagagattcggacaccacactaatttcttgcgaagtgtgacatatacacttactaattttgagatgtaaacttcttggcgtactatctagctggtgaagaaacatggtgaccttggcaaggctgtcctttgtgcagtgcaagcaactaatggagtttatgctactctgctctgctctgctctgttctctgaaagcagctcaggaattccgaatcagagtgatgtatactgggaccaaacaaatgttggtgagatcctggtccacgaagatcacgatgatgacctgctgactggatgttctagctatctttagtttcttcaattagtgaaatcaaattagatcctggctaatatggtcaaatccgtggcacgtgggtccacgaagaacacgtgggtctagctatctgttgtttcttcaatcagtgcagtcaaattaagttcaggttttccccgcaaaaaaaaaaatttaagttcaggtttgttctggggctcaggacatatgttgtggatggaagcaactgtatcaggacatattggatcaggacatgaaactgtaattgcag

SEQ ID NO: 6 - protein, 495 aa, Aegilops tauschii'PI511383'
MAGVLDALASYVTNMLTEMAKEEVAMLIGVSDGIKDLSIKLGDLKNFLADADRRNITDDSVRGWVGELKRAMYLATDIVDLCQLKAMEQGQTKDRACRCLNPLLFCMRNPLHAHDIGTRIKLLNQNLDDICKRGSSFNFIKLEAYQDQKTTRSPATDRKTNSLIERSGVVGEKIEEDTRALVEVLTREAVGDKSGRLIVVAIVGIGGIGKTTLGKKVFNDEAIEGKFTKKIWLSITQDFTDVELLSTTITAIGADLPGGGGAPDKALLVDALKNAIKDKKFFLVLDDLWDVDAWNKHLMTPFSYGGPGSRVLITTRHDTVARSMKAFHPYHHVDKLAPQDAWSLLKKQVVTGEENEPEVDMLEDIGLQIIAKCDGLPLAVKVMGGLLCKKEKTRRDWQDVLNDDMWSVSQMSKELNYAIYLSYEDLSPYLKQCFLHFSLKPKKTVITDTEMVSMWVGEGLVEGDTYTRSLEEGNKYYKELIVRNLIEDRLVEEED

SEQ ID NO: 7 - DNA, 2609 bp, Aegilops tauschii'PI511383'
gcagctccacctaccgcagctggccggtcgtcggtccttgcatcgcatccaaggcgacgccggctccaccactgccgccaccactgattggtaccttaagctcccgtgaagctacaagggaggaggccccctcgcctcccatccattgttcctcaacagcttgggtgccgagctcccccaccaccacactagacgcgctgggattcattggatccgctccagcgagcgagccggattcagttcaccgagattatattcacccttcccgtctgccaactgattacctcccttttcccattctaccctgggtgaccactctgctcactctcactctttctttctcctctacgccggccgtgcacagcgcgacgccgacgaccgcatccccccgacgttgccgcagccgccatacaagtagaaggaccgagatggcaacctctcccagctttgtgctacaccgcaagtactaggagcattgctgaatgccggatatagatccccagatctaggccaagggtctcgctttctgctcactgttacttctatcatctctccaatcgatccaagttccagctcaagccactggaccctgcaactacttgcgagacagcacgggatatctatctctgcaacaagatccgtctctcatctctctagtcgattcaagtactagttcaagcgtgagcaaaccctgcaaccaatggcgggggttctggatgctttggcatcctacgtgaccaacatgctcaccgagatggctaaagaggaggtggccatgctaatcggcgtgtctgacgggatcaaagacctaagcatcaagcttggggacctcaagaatttccttgctgatgctgataggaggaacattaccgatgatagtgtgcgggggtgggtgggcgaactgaagcgtgccatgtacttggccactgacatcgtcgacctatgtcagctcaaggccatggagcaaggtcaaacaaaggacagggcgtgccggtgccttaaccctctgctcttttgcatgcggaatcccctccacgcccacgacatcggcacccgcatcaagctgctcaaccaaaatttggatgatatttgcaagaggggcagcagtttcaatttcatcaagctagaagcctaccaagaccaaaagaccactcggtctcccgccactgaccggaaaacaaattcactgattgagcggtccggtgtggttggagagaagatcgaggaggacacgagggcacttgtggaggtgcttacaagggaggcggtaggtgacaagagtggtcgcctcattgtggtcgccattgttggtatcggagggattggtaagactaccctcggcaagaaggtcttcaatgatgaggccatcgaaggcaagtttactaagaagatatggcttagcatcacacaagatttcaccgatgttgagttgttaagtacgaccatcactgccattggggcagatcttcctggagggggtggggctccagacaaggccctacttgtcgatgctctcaagaacgccatcaaggacaagaagttctttcttgtactagatgacctgtgggatgtcgatgcatggaacaaacatctaatgactccctttagctatggtggccccggtagtagagtcctcatcaccaccagacatgacactgtagcccgaagcatgaaagcctttcatccctaccatcatgttgacaaattagctccacaagatgcttggtcgttgctcaagaagcaggtagtcacaggagaggaaaatgaaccagaagttgatatgctagaagatattgggctgcagattatagcaaaatgtgatggcttaccacttgctgtaaaagttatgggtggactcctatgcaagaaggagaaaacacgacgtgattggcaagacgtcttgaatgatgatatgtggatcgattggtggaagaagaggactagaccgaaactcctacggaacgagtttaggcgaaaggaccatatgatgcaaggatatacggatacctggaaagcatcagccataatgccatatacacttaacctgcagagattcggacaccacactaatttcttgcgaagtgtgacatatacacttactaattttgagatgtaaacttcttggcgtactatctagctggtgaagaaacatggtgaccttggcaaggctgtcctttgtgcagtgcaagcaactaatggagtttatgctactctgctctgctctgctctgttctctgaaagcagctcaggaattccgaatcagagtgatgtatactgggaccaaacaaatgttggtgagatcctggtccacgaagatcacgatgatgacctgctgactggatgttctagctatctttagtttcttcaattagtgaaatcaaattagatcctggctaatatggtcaaatccgtggcacgtgggtccacgaagaacacgtgggtctagctatctgttgtttcttcaatcagtgcagtcaaattaagttcaggttttccccgcaaaaaaaaaaatttaagttcaggtttgttctggggctcaggacatatgttgtggatggaagcaactgtatcaggacatattggatcaggacatgaaactgtaattgcag

SEQ ID NO: 8 - protein, 471 aa, Aegilops tauschii'PI511383'
MAGVLDALASYVTNMLTEMAKEEVAMLIGVSDGIKDLSIKLGDLKNFLADADRRNITDDSVRGWVGELKRAMYLATDIVDLCQLKAMEQGQTKDRACRCLNPLLFCMRNPLHAHDIGTRIKLLNQNLDDICKRGSSFNFIKLEAYQDQKTTRSPATDRKTNSLIERSGVVGEKIEEDTRALVEVLTREAVGDKSGRLIVVAIVGIGGIGKTTLGKKVFNDEAIEGKFTKKIWLSITQDFTDVELLSTTITAIGADLPGGGGAPDKALLVDALKNAIKDKKFFLVLDDLWDVDAWNKHLMTPFSYGGPGSRVLITTRHDTVARSMKAFHPYHHVDKLAPQDAWSLLKKQVVTGEENEPEVDMLEDIGLQIIAKCDGLPLAVKVMGGLLCKKEKTRRDWQDVLNDDMWIDWWKKRTRPKLLRNEFRRKDHMMQGYTDTWKASAIMPYTLNLQRFGHHTNFLRSVTYTLTNFEM

SEQ ID NO: 9 - DNA, 8844 bp, Aegilops tauschii'PI511383'
tgatcatcttcacacggaagaaccaagatcgttaacttggaaagataagttaaggatcacaaccgaaacatgcaaagctcttgcataccttcactctgctgtttcagtccctgtaatacatagagatatcaagccttccaacatacttcttgatgatgccttgacagcaaaagtgtcagactttggagcttcaaggtacattgccatgaatcaaacaggaacaacaactgcagtgcaaggaactataggttacttggatcctacatattattatagcagacgcctcacagaaagtagcgatgtttatagctttggagttcttcttattgaattgcttactaggaggaagccatctttgtatagatccaatgaaggcgttgggcttgtcatggagttcgttgcactacttgcagaaggcaatctatccgaaatactagacccaccagttgtagaagagggaggtagcaaagtcgaagacgtagctaatctagctgtgtcgtgcgtgaaactgagagcagaggagcgaccaactatgaggcaagtggagatggcgctggaagctctccaagcacgcaaggagcatgtcatgggtgatttgatagaagaaacaaacgggaagaaacatgcagcaccaaattgtccatcgactagcaaacgaccaaagggaagtggagcaagcagatgctatagccaagaagaagaggtggtgttatccgcaacattccctcgatagttttgcttgcccggaagtgatttttagtgatgttgtattctttctactatttggaatgagcgtgtgctattgtatgaatatatgagttacacataactctagtgtattatttaaaataaatttgaatgcacccaactctgttgtgctaattttgcatgttgtcgcgcaatcagcatttggtcttgatgatcgacagttcatcactagtggaaaaagtgttagtcacaatttttgttggtggcgcaccgactcctaacaacggtagtactattttttccaaataatggtggcgtcggacaatttggtacgacattgatttgagcataccgctggcatagaatttttctcgtaccacataggcattttctgagtttttttccgtgtgctttcgttttctatagcgtggcccattaggcatacgacagcggtatccattaggcccacgcgagcaaaataaaactaccctatccagtaaagatcagtgtaggtccgattcactaacctatcattttcgcctcttcttcatcccccttctcgaccgccccgccaccgccactgcccgatgacgccgctcttcgccgccggaactgcgcggccgccgccaactccggcaaggtgctacactgtgtcatgtttggtcgataggtgctacgcacgacaaatcctttgcgtctggatggacgagcgcaggacgatagcgtcgtcgggcgtcgtggtggcatcgacggaccggtaaggatgatgcggatctatctcctgaagatgggtcagcggtccgatgatgatggcggcttctaaaacgtgtgcatgtgttgtacgcattttgtctgctgcgccggtgttagttctgatacattatgtggatggatcggcgacgacactggttttagatatgggagtgagagccctccacattatcgagttttttagatgtgagtagtggtttcgggtggcttgatgtatattcctgttcgacctttgttgaataataaataaagatgaccgtatgcatcgattgatgcagaggccggtgttttaacctcctttttgaaaggaaaagtactatgttagtagagtgcttagctgattaaggatgaaaactgcaatagctccttactttccctggtaaaactacaaatatcacaaatgcaaacccacccatcccggtagcctcgtcaaattaaaataaaaaaaaatataagaaaaggaaaatgcgaccggcggctagcagctccacctaccgcagctggccggtcgtcggtccttgcatcgcatccaaggcgacgccggctccaccactgccgccaccactgattggtaccttaagctcccgtgaagctacaagggaggaggccccctcgcctcccatccattgttcctcaacagcttgggtgccgagctcccccaccaccacactagacgcgctgggattcattggatccgctccagcgagcgagccggattcagttcaccgagattatattcacccttcccgtctgccaactgattacctcccttttcccattctaccctgggtgaccactctgctcactctcactctttctttctcctctacgccggccgtgcacagcgcgacgccgacgaccgcatccccccgacgttgccgcagccgccatacaagtagaaggtgaggacccccttcctctcctcttcgtcctagccagcggatcctcagatctgagctgagtggggccgcagcaagctcagactaaattgtttcttacaaatctttgagatgatttccgtaccacgtatagaactcctaatttctcagcagaagaaatcaccgggttctgggtttgcgcacaaagctttgattttgttttgtgctgtgctgtgaaaattgagctcagatcttcttttagtagcctgtgatttgtgcagtccaatttgctgtgcggtaccaactaagctcacatctttttagtagaaagtacctagtagtttttagagctttgctttgcaagtagtacactagtactacaaattaagctcacacattatattattacagaggctctgttttgttcagtactacaaagcttagattttgatttctgtactacgaatttagctcagatcttttttctgaacagcaagcttttaatttctgcaaataggaccgagatggcaacctctcccagctttgtgctacaccgcaagtactaggagcattgctgaatgccggatatagatccccagatctaggccaagggtctcgctttctgctcactgttacttctatcatctctccaatcgatccaaggtaattcatcgattgcagcagcaccaccctctatttagtgtgcactttcttttgtgtgcaatccatgcttttcctttacaacgaattgttggtagtctctgctgagtgaatctacatgaccatccttcttttccattttttttgcatgtcactattgatgtgtgaaaggtagtaataaagaggactcattttgtgtgcatcctttgttttcagttccagctcaagccactggaccctgcaactacttgcgagacagcacgggatatctatctctgcaacaagatccgtctctcatctctctagtcgattcaaggtacatagctgaatccagctacacaacacttactctagttatttttcttttttgaaagagctgatcgtgtgtctttccatttcaattgttggtgtttgttcaaggtaatactatatcggttttatttcgagccgaatttctgtgcactgtctttgcaagccacattttcctttggatttgttactagcctctagtgagtgaatctgattatccttcctgttagcatgggattgttgatgtgaaaaagcgaggtagtaatacaaaggactaatttttatttccatgcttcttttcagtactagttcaagcgtgagcaaaccctgcaaccaatggcgggggttctggatgctttggcatcctacgtgaccaacatgctcaccgagatggctaaagaggaggtggccatgctaatcggcgtgtctgacgggatcaaagacctaagcatcaagcttggggacctcaagaatttccttgctgatgctgataggaggaacattaccgatgatagtgtgcgggggtgggtgggcgaactgaagcgtgccatgtacttggccactgacatcgtcgacctatgtcagctcaaggccatggagcaaggtcaaacaaaggacagggcgtgccggtgccttaaccctctgctcttttgcatgcggaatcccctccacgcccacgacatcggcacccgcatcaagctgctcaaccaaaatttggatgatatttgcaagaggggcagcagtttcaatttcatcaagctagaagcctaccaagaccaaaagaccactcggtctcccgccactgaccggaaaacaaattcactgattgagcggtccggtgtggttggagagaagatcgaggaggacacgagggcacttgtggaggtgcttacaagggaggcggtaggtgacaagagtggtcgcctcattgtggtcgccattgttggtatcggagggattggtaagactaccctcggcaagaaggtcttcaatgatgaggccatcgaaggcaagtttactaagaagatatggcttagcatcacacaagatttcaccgatgttgagttgttaagtacgaccatcactgccattggggcagatcttcctggagggggtggggctccagacaaggccctacttgtcgatgctctcaagaacgccatcaaggacaagaagttctttcttgtactagatgacctgtgggatgtcgatgcatggaacaaacatctaatgactccctttagctatggtggccccggtagtagagtcctcatcaccaccagacatgacactgtagcccgaagcatgaaagcctttcatccctaccatcatgttgacaaattagctccacaagatgcttggtcgttgctcaagaagcaggtcggtacttcccaaaactcaatataatacacgtcgtttgggactacactgttaagttaatttgatctacacttgcataagtctaccaatctgaaatttatatatttataatgcttccttgacttaaatttcaccgtaacacgagttcatcaagtttgtatatgaaattaggaagatattaaacaatattttcatttgtatgcatgatgtacggcttctcaatttgtggattattccggacttaagtttagcaattatcagggattgcatccagcttctcaattagtttctacttgcaggtagtcacaggagaggaaaatgaaccagaagttgatatgctagaagatattgggctgcagattatagcaaaatgtgatggcttaccacttgctgtaaaagttatgggtggactcctatgcaagaaggagaaaacacgacgtgattggcaagacgtcttgaatgatgatatgtggtcagtatctcaaatgtcaaaggaactaaattatgccatatatcttagctatgaggatttgtccccttacttaaaacagtgcttcttgcacttctccctcaaaccaaaaaagacagtgataactgatactgaaatggtgtccatgtgggttggtgaaggattggttgaaggagacacatatactcgtagtttggaagaagggaataagtactataaggagctaatagtaaggaaccttatagaggtagatacaaagtaccctagtcaacttatttgcaacatgcatgatgttattcgctcatttgctcaatttgtggctagggatgaaacactagtaggtcacaatggagatactatcaaaacaaatcttagatcaccgaattatcttagattatccatagaaacgaaaggagtgggatccgatgaatttgagtggagatatttaagagagcaaaaattgcttaggtctctaatattaactggaaacctcaaaagtcagcctggggattcgttgactatcttcccaagtctacgtcttttgcatatagaatcagcaaatattgctgcactagttgaatctatgtaccaactcaagcatttgagatatttggcattaaagaggactgatatgtgtagactaccagagaacatccatgagatgaaattcctacagcatattagccttgaaggttgtgaaagtttcatgaaacttcctgatagtattatcaagctgcaagggttgagatatcttgatatgggtgacacacgtgtaagtagtattcctaggggtttccgagctcttacaaatttgacttcactatttgggtttccagcctatattgatggtgactggtgtagtctggaagagttggggtctctttcccagctcaatgaactttcactacagagcctagaaaatgtatctagtgccttgttggctgaaaaggcaagggtaaatgcaaagaaacaacttaccgtacttgctttaaaatgtggtggtagagtgggacatgggttggtccaaggagaggtctctgagtctaaggaggaggagcaaataattgaggcggtgtttgatgtgctctgtcctcagccttgcatagaacacatcagaatagaaagatattttggtcgtcggctcccaggatggatggcgtccacagctatggtgcccctcgagagcttgaagattctatgcctcgaacacctgccctgctgcacccaactcccagatggcttgtgcaggctcccgtatttggagtggataaaagtgatgaatgctccagtaatcaagtgtattggtcctgaattcgttcaacagtacaatcagctgcaccgtccttcatctcagttggctgctacgtttcccaaactccagatgttggaatttcacggaatggaggaatgggaggagtgggtttgggagacggaagtgaaagctatgcccttattggaggaacttcgtatcacttcttgcagactgagccgtatgcctccaggacttatgtctcatgcaatggctttgaagaagctaacaatatggagcgtccaatgtctccactctctagagaactttgtttctgtagttgaactcgaattgggaaacatacctgaactggccatgatctccaatcttccaaaattacaaaaacttacaatcgagtgctgcccaaagctcgagatgctgcaggagatggctgcactccggagactcgagctgaccattttcaacagcgaaaatcaacttccggtctacctgcagactgtgaagcctagtaatttgctgctgacctgcaacctagcggtactcacttccatggctgagggtgaatctagctccgagtgggacaagttcagtcatatcaaccacgttgaggcttatgcagaggatggagaagatgagaagaaatggcacgtgttctacacatctgaatcctgcaacatagagacaaatattcatcaggtaatactttggtctctccctctttcaatctagctaataataatattcttccttattgttgtctgttccatgcatatctattttcatcagtatgatataggatagctgaatatatctcccactgtttttgttttgcttgccaggatcgattggtcgaagaagaggagtaggctgaaactccagccgaacgaggaaggaccatatgatgcaaggatatataagtatgtctgctgttacaacttcaactagttttgagatcgaatccatgaagggatacggggaaaagcatcagccataatgccatatacacttacctgcagagattcacacatcatactaatttcttgtgaagtgtgacatatacagttacgaatttagagatgtaaacttcgtggcggactatccagctggtgaagaaacatggtgaccttggcaaggctctcctttgtttagtgcaagcaactaatggagtttagactactctgctttgctctgctctctgaaagcagctcaggttgcaggtcctctgaagcagctgcgtttttctttttcttttttcgcgggtgtctttcattcgttctctggaaaactatgtttatttctgatagatcaatcaatagtatactggaacactaaatactgttagaacaaacccaatcaaaatgtactaatgctctgcacctgtgagccaatcaaacggatgtatatcaaagagaggcatcatattattgaggagccatcggagattttctgaatttgcccagcttgaggatggatctgggccgccgccgccgccagcgttggggccgcagctctgtacgcgatttgggattgaacgatgaggccatcgagaccaaattagcttgcagggaaggacctttttgcaaattatgcgcctaaatctgggccatcattttcctatccggtggtccagatccactttttcgatttttctaccataagcatgttttctgttgtagttgctcctcaacagttgtacgtattttgatggtagatggatcatggatggatgcataaggctggtcatagtgggaagtatcatatactagtatcatgcatatgatactagtgtataaactacatccatagtgcatagtatcatagattagtatcataggtggtctcatttattgccatgcatgacacatagtagcattacattaattatgttacggtatctacctatgttactataactatctctctcttctttaattgcctgccacataagcatgtttgcgattcccaagtgcatgatactacttatgttacttccactatgaccagcctaatgcatcttcacaatcatttggcatcactggccgccggccaccgtttttactccattattttttgttcagtgggtagtaaggaaccagtaacaattaataactggttaatagatgcatggatctgataaataagccaactatttagcaactttaggtgctaacttattaaataaggtgtgcttagcaataacaggttaagcacctatacattgaggagttgagttgctaagatatttaatgcacttaacatctcatttaagcacctttgcatttgaagaggtcaaagtgacagctagcttactcagcttaagataatttgagttccggaaaaggttttcgtcccgctttatataattcaatcgaccgttcacatgcaggactagctgtaca

SEQ ID NO: 10 - DNA, 39535 bp, Aegilops tauschii'PI511383'
tgttttaagatcaatgacctttttaaatttcgcggccctttttcaaagtcatgattttttttcaaattcatgattttattagaaaaatataatgaactttttcattttttcgaattaatttatcaaattcgagtattgtttttcaaatcgatgaaatttttataaacttgtgagcgaatccatgattttttaattttaaaaccgggaactggtttttcagttaacaaaataccagcagaagagaaaaccgagaaaatatagcgaggaaacgaaaactgatgatcacaagcggtgaacaggaagtggatgccgaggtgcttgggctgcggcccagtaaggcaggtgtgagcaccaacttattttcctggcacataaggctccaaggaggaaaaaacttcatgattttgtaggaagtttgtgaaaattggaaaaagttcaagaatatgaataaagtacgcgtaagggaaaaagttcactgatttaaaaaacgaagttctcgaatttgacgaaaatgttcgtgaaattgagaaaagttcatcgattggggaaaaaggttaacaattttacaaaaaagaattacgaagtaaatatttttttcataggaggcatcccgactggatcggcccattattgcacaagaaaaaagggaaaattaaaatatcaattttaaacacttgtttaaattatgattttaaatacttcttgccttcaaacctggcatggatgcctatcatgtgcatgcccacctactggcaaaagttgatatcatttcataaatgtccaaaaaactagcatgttcaatgtagggtgtcggagtaggtcagaatgctccgtttgagagcacattgtttggtttgctaatttgtttacattttcaggagttttctaagtcaaaaagggcgataaatggccgaatgggttggaactagcatacattgtcgaaaatcgttcaaacatgacattgatgcctaccatgggcatgcttttcatgcatgtccaaaaatagaacatgttcaacggagggtgtccgagtaggcgagaagggtccatatgagagcaagctttttcggaatcgcccagtaaccccatttcccatgagattatatgaacaattaaaggcgccatgccaagttgtttgagttttggataatatttgtattttctggagtttttttgttgaaaagttgctgataaattgccggacgtgacgcaacttgcatacggtgttgcaaagcgttcaaacctggcatggatgcctaccataggcatgctcatctgctggcaaaaggtaggatcattaaatttatgtcaaaaatagatcatgttcaaagtagggtgtccgtgtaggctagaaaggtccgtatgagaacatgtttttttggcatcgtcaaatatccctaaaaattttacatgagcatatatgacctatttaaaggcaccatgcaaagttattttagtttggacaattgttgcactttctagaattttcttgatgaataatgactgataaaacagctggacgtgatgcaacttgcatccggtgttagaatatattcaaatcaggcatggatacctatcatgggcatgcccacatgctggaaaaagttagagtcatttcatgtatgtctaaaaatatatcatgttcaacgaagggtgtttgcgtaggccagaaggggtcgtatgagagcatattttttcggcttcgtcatatgaccccaaatttttcccatgctcttatataaccaattcaaggcaccatgccaagttgtttgagttttcgaaaaatcatgcattttctggagttttctcggtgaaaaagtgatgataaatggctggacgtgtcacaaggttcaaacggtgtcagaaatcgttgaaaccaggcatcgatgtttcatatgtccgcgccaggctgctgtaaaaagttggggttatttatccgtagtccaaaaaaccaccagttgagagaagtgtgcttactaagccagacgagtgcatccgtgagcatggtgtttgtattttccgctaatataattaacacgaaaaaaaatgtcctaactatttctttaaatttatctacaattttagatgcttttgttatttgcaatttccgtcattgtcaatgaacatgaactttaatttgtgcaaagtgcacacatttgccaaaattcgaaaaaagaaaaaagaaaaagaaaacagaatataacgaagcaaaacccggttttttaaaagatggagaatggccaaaaatttcacaaaattacatttgccacataagaagccaaaaagaaagcaagtgttcaagttgtgttcaaaatgttagttcctatgtttgcacgctcctcaaatatctttaaaattgttcaaaatgttgttcaaaaaaatgttcttaacattttgaactaacataaccatttaatttttttgttttcatgctttaaaaaaatgttgttcattgtttttaaatgttcatgtcttttttaaatgaaaattttaatatgtgttcaagttgttcaaaacattgttggattttcagaatgttcgtgcgcctagttcggaacccctcgtccgtgggcctgctgcctcgttatcttgcagcattcaactgacgttggtgctaatttggcagatcatggacgtggcagctccttcaatacattagttagcaaaacagccatttatccctcatgatcatgtaaagtggaacgcctttatccctaaaaaacaatcaaagcagccactcctagtcgattattccccttttagctgattttgatccgtttttgagggagaaaagggcggcgtgataggcttccctccccattcgattattcccctcgaccaatctacacatgcctagattacgctgcccttccttagtcgccctatgtacacctggacctacttttttttaaaatttacacctgggcctttttttaatttacacatggacctactgggtacatgtgttttggttgacgggctcaataaactcggacggaaggagtggttcgtaaatttgcacgctcctcatttttcacaaacactagtcagagccactcactctcacgtgcacagaggtccgtggtttgattcctagagggtgcatgcatacttattttgtgaacttttactccggcgggtgagtgatgtattttaataaaagaccatcttaccctttttaggggagaccatcttaccctttagtatgaaggggtatgaagaaatctacttctttgaagtgattaggaaggttgtaccaaaggagaagtgacattaaaataacgtaaaatgggcggggacaaacgagactatgagaatgcaccaaaatgaaaaaaacaggcttaccggtcataattttgtcggcaggctggtggacgtgtagcaggacgagcttgtcgccaccggtaaggaggtttcgagcggcccacatgaggtttgacctgccgtcctcttcatccttcccgacagccacatacaagttccttcctcctccgccgccaccatcctcttcgcccttccataagggcacatacatccttcctccttcgccatcatgctccaagttggcggtggtctcctctttggcacaagcaccgacaccggcaccgaggctagcgcttatgtcggactcggtggacgacctccgggtacgccacatcttggcccagtaggatcggttcctcagcttaccctcacgagcagtgtagctatacatcaagccgccggaagatgatgatgatggtgatagtgatgatgatgccggcttaggcttaggcttacaaactcttgagaatctgctccgccaagctcgtcaaacagatcaaagagactgagaaatttctcccaagaacccttgacccgaagattcgaaccctcgaccaagctggccaaagagatcaaactctggtcaaagagattcgaacacgcaatttctcaagcatgtgttttctgttctcaagtgcaatttcaagcttacaggacgcaactgacacacattgtatagtttttaggctgtcaaatgcatttttttctgagcaaaggaagcttcacgaaggaaccagagttttctttttggcaataaaaccccctctatatttggtgcacgggtcgccggttagcgaccacgcgtggacccccccccccccccctacacacacacgctggcctttccatgggctagtttttctttttctttctttcgtgtttttctattctttttattattattttttcatttttctagttttttcagtttgcaaaactcttttaaatttatgaatattttggaaatcatgcacattttctgaaatgatgaatttttttaaattgatgaacatattttcgaaaccgtggaccttttttttacaaacttgtgaagagtctcctaaatcccgaatgttttttgaaatcatgaacatttataaaattcgtgaagaatttgtcaaaatcatgatcctgtttttaaaaaattcatgatcattcattttttgaaatgatgaacgttgttcgactcatgaatattttgtaaatttatgaacaatttttcaaaattgtgaattgtttgaaaatttgtgcagattcttttgaattcacgaacattttttaacacggcactgccagccacctgagcaagcccgacagcatcgctcggtggtggcaactggagagcgcacagggtgagggggccgagaaaagtgtatcggaacgctgcctgagtcgcccgacaaaaggacgacgcgggggcatttctgtttttttaacacggcacattcgaagtcactcacatacacgagcatacaatcaacctacaaatgtgtgcacatacacaccttacccctatgtgtgatattcaatatgttgcattatctagcacatatcatgttcttatttctgaataataggaccggcagcgtgcacatgtccacgtacagttcagtagcttcacttagttagtctgtaagtagattcagttagttggttagccagatttgctcaattgatcgcttctagggatgctaggatcgttacggtttatgcgggcagtgtagttgctcgatttcagcttggcatcgtgggatggcacgaccagtaggccggcttgaaacatgggcgtctcccgtgtaattcgtcagccgtttgagctggctacaaataacagaaaagcagagaaaaagctgcagttcagtgagcagcacaaaaacttctgtgagagtctctcctaccacctctcgcaaagctcggtcgttagtgctaggcaacaacaatgataacctccgagagactgagttgacacatgcttttgagattgacaaagttgccataaacgccttcgtagtcgatcagatcgtctcatccccacttaacgcacatcaccggaacaaggtatgtgagaaccaatgtcatgtctaggacttgaaatctggtgggttgagaataccactaccctcataaccatcataccgcagcttggttcgccgttttttgtttgttgatatatgttcccccacggtcacaatgttttggtacaggaaaaaggtaagaatactcaatagtagaatgttgtggagaagtggtggcagaggggccgtacatttccttgtaacatgcctctgccagtagtccgtcctctcatcgaatcatcatggttgaacatagcttactattttcttgataatcattatcttcatgttcaactccaattgttcctacagaaaatatattcagacttagcacacaaatgaactatgagtgaactactactgaagaaacaaggctcacagtttaaggagtgacaacgtatctgttcaacaggcatgactttgctatttgccagtgtgttttttatgagtgtgcgttagtgttgcctgtgtgtaacccagccatgcagaaaccgggtgcgtgctcattgcgtttgtatcatcttgatgcttcattttgagtgaataaaatccacccattaaaaaaaataagcattgatgttcctggcctagcgggagaaagagaggctggaatcaccgtcccgacctttcagggcagaagaaaaaggttatttgaccaacggttcttactcttagtcatcaaaactctgtgcgggtcccggggagactggcctagtccaagtcttcacatataagtgagggacatgtttgttttccttttatttttgtgagaacacatttttgttttgacggggcacaaaaagccatagacctgtatactagtccttttcgagactagtctatgttagaatagttagaatgaagcatcataaaaaagacaatttctgatgcttcattctaactattcacgaggcatttctttatcttttttacacaagccacaaaaaacgtcgtttttcaccgaaaccttgtgaacggacataaaatgtccggatatacacgcggggtttttgttccgaatttttcaacttttcaaaatgtgtgttttcgacaatgggtgcatatgcacctatgagcaaaaaagccgcgtccggtgaagtttgcatatcatcttctttacaagtatataaagcatacaccaaacaatctggactcactaacatttccagccaatcagataatttgcataggtctggctctagttaagtgaagttgtttgttttaaaacacaaaacatattcctaaaatatctggactcggtctcatttccagccaatcaaataagatggatatgtagctctggatccatcaatatgttgagggctagaaaagccgtgtggaccactcaaacagacgcttgctggctaatgttgctttcaacagggatttgaccaaatccgtacgaaaaatcacccaacctcgtgcgctctattaattttttattctgtctttcgtcgttgggatattaaaccgtcatttattttttcttttttagaagtctcgtatgtagctatccgaatgactcatgcatttgcaaagctgcctaggaaatgacaaaatttgcgaatgagttttgttattttctacccacatgaatgttctcaggaaaatagatattttacagatttgcagttcactcaacacattttcaaagagggcctcgcacaccttagcgttagcgagtgatatagatgcgcacacctggcttactcctgcatcgtagcgcataactgcataagtacaccactggaattaggtaactgtagcgacaagtcaatccgtcctgtcctgccatacataatgctaagcagctgcgtatccattgcggcagcggtggtgctgctgctaatctcggcaccggcggccgcagcagggcctccgccgatgaagatagggatgccgggctgcaacaccacctgcggcaacgtaagcgtgccttacccgttcggcatgggcccgaagagttgttactggccggggttcaagctcacctgcgacaacaacggaagcaatctcccgcggcttctcctcggcgatggaagtgccggcattttcgaggtcgtcaagatctccgtggagaacactacgatgcacatcatcagccacggactgcaagccatcaacatgagaggcggctcgggccggtggagcctcggtgatgctgagactgagagcatcggcgccggcaggttgccctacttgctgcacccggattcaaatgatttcatcctcacgggttgcaacgtgcaggcgacgcttctggggaaccgcagcctcgccagcggctgcgcttcgttctgcccggcttttggtgatggtggtggcggtaacctagtttattctgggggaaaatccaatacctgctccaacatcggctgctgccagtcgaccatccaaactgccagcgcgtcctacggcgtggagctcaagcggctcaactacagcggcgtgtacagcaatttcgatttgcccgtgcacgtgctcatcgccgaggtgggttggttcgacttagaccacaatcgggaggtggttatgaacctgtactgggaggaaaaccaaaaagaaaatctctcgcggaaggctgatcggctcagggtccccgtgattctcgcgtgggcattggcacacgaggcagcagtgaactctggccatttgcattgcccagaccacgcagcccggagcatatgcaagagcgcccacagcaattgcagtgtcggagactttcaagtcagaggctattcgtgccagtgcagggagggctaccagggcaacccttacctcaccggaggatgccaaggtgagtttacaatttttttactgaattatttgcattgctttccatatgtgtcacgtggttatttttgttcgtggacatatacacagatatcaaagagtgcgatcaaaaagaaaaacatttctgcttcggggactgtgaggaactgccgggctcgttccagtgccggtgcccgaacggaacgcatggcaattacacaaagcccggtggctgcatcatcatcgagtctgaagacacaatcggaggtactcctagcctgccgattactagtgcgtgcaacaggagacaatggaacaattaatgttcattagttaattatctcgctccatttatatattcttgataaaatagtactagtagtaaatgtgtcaattgcttttcaggtcataataacttgggtttaatcattggtctctcggtcgctagtggcccatttattctacttttggttcttggtgcaatcctaactatccgtggttttaaccaacgcaaggcgaaggcgctgagacagaagttctttactcaaaaccgtggccaactattaaagcaattggtttctcacagggccgacatcgcagagcggatgctcatctctttagaagagctagagaaggctaccaacaattttgatcaagcccgcaggctaggtggaggtggacatggcactgtctacaaagggattatgttagacctgcatgttgtggccatcaagaagtcaaatattgtcgtgaggagagaaatcgacgagttcataaatgaggttgccatactctcacagatcaaccatagaaatattgtgaagctccgtggatgttgcctcgaggcagaagtgacgttacttgcttacgagttcatttccaatggaacactcgccgaccatcttcacgcggaaaaaggaggatcgctaccttggaaagataggttaaggatcacaagtgaaataggcaaagctattgcttaccttcactctgctatatcagtccctgtaatacacagagatatcaaaccctccaacatacttcttgatgatgccttgacagcaaaagtgtcagactttggagcttcaaggtacattattcctgtggatcaaacaggtacaacaactacggtgcaaggaactatagggtacttagatcctatgtattattatactggacgcctaaccgaaagtagtgatgtttatagctttggagtccttcttgttgaattgcttactaggaggaagccatctctgtatagatcttccgaaggtgatgggcttgtcatgcaatttgttgcactacttgcagaaggcaatttggcaaaaataatagacccacaagttatagaggaggggggtagcgcagtgaaagaagttgctactctagccatggagtgcgtgaaactaagagcagaggagcgaccaaccatgaggcaagtagagatggcgctagaagctctccaagcacccaataagcgtgtcggggctgatttgatagaagaaacagatgagaaggaatatgcagcaacaggctatccatccaccagccaacaagcaaagaaaaatgaaggaagcaggtgttatagccaagaagatgagttcctgttatctgcgacataccctcgatagtttttgcttgcttgtaagtgaatttttagccatggtgaattgtttctgttattgtaaatcagtgcgtgtttttatatgaatatatatgccgaacagaacttaagtgtatgcttcaaaaaaactgaatgcacccaactatgttgttctaattttgcatgctgccctgctctcagtcttgatgatcatctatatatccatcttccacacgtactcacaagactgaccaagacactatccatcatttcgttgcacttatacgtatttattgatgtgtcgatccttgtctccattaaaaattgtgcaacttgtggtagtagaagcaaggtagccgctcgggtgttgggcatcttatttaaccattgaaccccgcgatgtcatttgatatctcagtatcgtcttgggaacattgaactgcacaccccagaatgcaaactataccaacactatggtacagtgcatgtaatgcaacaattggtttcatctccacgcaaaaattggaattaaagcaaacgctgcacatgcatgcatgctggttgctggccctacacatgtacatagaacctctatgattcgagcgtgtgatcagcagggactggtgatgagtccaaatctcatctccgtgttcaaataggtacatggcgtgtttcggctattgaggctcccagcagcaaacacactcgagtcaagtttctatgggtgttctcattgacctgtccctcaacaatccacttctgtactactaccgtgcaatataacccatctgactacaacatgtgggttaccattgtttcattctactctaattgcccttctaactaccctgtaattcccctgtaaagccccatgtgtctagcattgctctcttcgcagtcttagcaaatactatttactccgtacgtatgcgcccatgcagagaccggtaaaggttttaactctcaactgctaacaacgtactctaagtaactctcagctgctaagagcatctccagccgtttgaccgcccaaggcgtcgaaaaagagcggcctaggagcgagccggcgctagatcggcccctggggttcgtttctccccagccacgcccccaggtgcccccccccccccccaaggcgccccatattcgaactccatcgttcccgctcaaagaaaagcgatcatcgcaatagttcggcgattcagtgccacagttcggtgattaaataaaaggacacgcagtagttcggcgtacagaaaaggaaggacgcgggaggagtacatcaaacgtcgagctcaacctccggcggcggcgtcgtcggcgtacgcgggctggaaggagtcggcgcggcttctgggctggtcggcatggcttctgtgctgccgggcgcggcggaggcatcgtcggtggggctgggcgtcgcggaggcatcgtcggtggggctgggcgtcgcggaggcatcgtcatcagctgccgggctgggcagcggcggcggcgtcgccggtaactgattcaggatgtggccgcgctccgccaagaaccacgccttgagcttctcgtcgccgctttggagcatgtcagcgccacccatcaagaaggcgaggtcgttgttcctcttcttcgcgtattgagctttgagttttgcggcgccgttggtccggagcaagtcgagtttgacaacgttgttcgtcatcaaaacagcccacctcgcctcagttttctcttctcgctgggcggccctggtcttggcgtcggcgagacaatgttcgatggactcctgcacgcgcgaggcagccgactcggcgtatttcgccttcttggcacctttgttgccgtccggttgcccgtcagccgcgcccgcggtcggcgcgtccggcttatacgtctctttggctttggcgagggtgcgcgggacggctgcccatttctcgcacctgtcgatccgcctgaagacgtggaggtacttgaactctgcgtcactgttgtcatcgcggaacatggcgaacatgcgtagcagctgcgccgaacgaaagaacatcagtcggcgtgctcggcgcgcacgaggcgaaagtgtgcgcgcacggcggaaggcaacagtatgagatacctgatcctcgacgctgatgccgctctccgggcgagccgcgacctcctcgacgatcccatgccatttgttgcacgccgtttggatgagcccccaatggttcgccatcaccgtcgccccacgcttcatgtgcacgcttttgaagtaggggtcgacgagcttccgctcgtcgaactcggccttgatgcggtcccaatacgtctcgatgctctggttcgtgccagtgaccgggtcgaggcagacaaccttccacgcttcggcgaggcactcctcttccttggacgcccacttgatgcgtggctcgccgggcttggccgccttcttcttcctcttcttcttgcctttactcgtcggcgccggttcctcctcctcctcttcctcctcctccggctcttcctcgccgtagtcgagctcgtcgttcatgtcaccgaggtcaatcgagtcgtcctgggtagtgaacccgggggaagcggcggcggcggccgagccggctgcgatgatgtcctccatgtcggcctccgtcgagtcggcgttgccgagatgcatcaaggatgcggcttgcgagtagagaatgcggcgaagaggtggcatcggtgaggctgcgtagtccggcggcgagtaagtgtatggcgggtactgcacgccggcgaatgctggcgagggcgtgcgctggacagggcgcccatggggaaggtgatgttggggttgaagccaccatgggcgtccccatcggcatagcccggcgacgacgtgctccatgggtgcggcgacgacgagaaccctgccggagagccgacgctttgctggctccaggccgcgtatgggtgcccaccgggtggattcatcatcgccgcgcacgccgcctccgcttgttctgccaccaccgcagccgtagcgtgcgccgctttttccctggccttcttggccctgttgcgcctgtcggcggtgacgacctcccggtgctccacatccgccttccactcagcgttgctgatgccggggggcttggatagcggcgccctcggcttcctttgcttctgctgggcggcggcggctgtgggatccgtcgcggcgcgcggcatcacgtacttcttcggcggcatggcgggcgtttggcgggaggagccgagcgtttggcgcgaggagccaagcgtatcagattgggatattcttgatcgatttggtcggatatgtagaattggtgggaggaatggagaagagatgggagcctagggggaaagcgggagaaaacggcgggaaagggcttcagtcgccgacggagcggccccacgccggttttcgcttgtgccggcgcgcccaggcgacacccggccgcttgggttcggggcgggatcgccggctctgtatttcgcccaaaccggcgctaaacgagatcctagggtcgtgactgggccgattttcggccaccggcgctaaaaattcgcctggggggtctgttggaggcgcggctggagatgctctaacaacctactctaagtgctccctgtccaaggaacccctgcttctcctccggctgtgtcccgtgtgagcaatgtcgtcctcacctccggcaaggccctggccaaccgtcgcccgccacttgttagaataaatctgaggcataccgtcgatcatccgagaactaagcaatcacacgaggcacgacgccgagatttgttaacgaggttcaccgatatggctacatccccggggcctgactacaggcgctcctccccgtgacaccgtcacaataccgcacccggtcgccctggacaccggcacatgctgccggcttcccctgcgttccggtgctattatgttggcataggttacatcgtgtgtctacccccggtatatatgagaggcctaggatacaggtctcctatttggagactccatatcctatctaaacacaatgcaactacaagtccaactgtaacctaccttgtacacaatattcggcacaactctaacaagcgccatcctcgtctcgagatcggtcgctctttaacctgagcggctgtcaagcaatataaaaagtctgacacctatattcatttattctgtatattcatggtaggtggtgaataattggttgaccaccctcacgacatccttataaaaggaacaatattccgcggcaagtcccatagaaaattgacaaatattgtccagaactgtatgataagaattgttttcaagctgtatgtaaatcgtaggcttgagagatatcgggaattaatttaccagtgaggcgctcttgtagatactcttggccacgtctccgaggaacagcaacatcacgaaatgagttgctgtggttgtcttgctgtggggaaccacctactggaggatcatgggaacctgtagcctgatcttccgctctacgttggacagatccacaagtagtacctgaccaaattaccccatctcggcgatgatcaggttcacgcccttctccggtaggctgccgtcctgtggtttcagctccaccacataggacgcgtatcccatgagattgaggatggacgactcataggagccggcgttgcaccaggccttaccgccgtgacacgtgcctgtggccatcaattgcggtttccacttctttcatcatgttgagctagcaaagcaggtggcttctagtttctctatgttagtgtgttagctttagctagctagtcttcggaaggatcgatctaatcgctagcttagtatgtgcaagtctcccgaagcttgtacatacgcgtgtgtttctcggtctcggccaaaagtattaaatgtcgttttaagtccagcttaatatatttttgccagaattttccaatctattgaagcaagcaactgaactctattgcattcattttcctgttgtcacccaaattccctactactcaaatttgtgataatcatctatcataattttcactcctacccaaagagaccaatcaagacaccacctttgccaaaaaagaagaccacaatcaagatactatatgctatatttaattaggtggtacttcctctgatccaaaatatagtgtgtattagatttttttttcaatatcaaatcttgtaaactgtaagcaagttcatagaaaaataataatatcaacacctataatacaaagtcaataccattagattcatcaaatatatttgcacttgatttggtactccctcccacctgagttaactccctatcctttgtaaaagacctagttgctcacccacacacactccccctcaaccagccgccgcgacctcctgacctcgccgcccatggcgaggacgcagccgccgtgagcctctgccgctgtgccgccgagccactcgcccgcgcgccgccgccgcttagacaggccgcccccgcatcagccatccccgagcagcagggaaacgggcccaaccgccggccaccgcgatgggctttgccccggcggcgagggtgcgggagggcgggaaggagggaagggaaaatgatgcaacggaatattgtctgaataaagggaaatactaaaaactgaggaagcgaaactgaagaagacatacactaaagaaataaataaaagaatgaaggattggaaaattgtgtgcaaacaaactgaatactgacaactaagaactaagagactaactaagagatctttcttggttttcatcagttttctttgtgtcactgcttccattctttttgcattggtttttgtttttgtttcccttatttccgtttggttttcattcgttctgttctcatttgatatggaatgggaaccttgttttatacacaattaacacttattcgaatacatgaaacgttttctgcatacgtttgaaacatttcttgtgtaacatttttccaattacatcattaacattgtttttaaacatatatttattatttcaaaaaaattcatacacattctatgttttccgcatacatctgcaacattttttgtgtacacatttaacattttcaaatacatgattaacatatttcaaaacatatctttttttatgttgcttttgcctacacattgtaaattttttgtacacattagaaacatatttttgtacatgctcaacgttaacacatgattaacaatttttgaaacatttattatgtctattttttgcatacaaattgtacattttttatacactagtaaaaaaatacacgtctaacatttgctaaatatatgatcagtattttataaaaaaacaattttatgagtaattgttttgatacacattgtacattttctttatctatcgaaaatatgattttatacacctttaacattttttctatacatgaataatacatttttacatatatatatattttgatgtctaatttctaccatacatattttacattttatattaacattaggtacatttttcattcactttaaaaaaataatacatgcttaattgtttttcttattttttatgtctacttttgtcgtgcgcatttttaaattctcatatgcattaggaacatttttgtatatgcatttaacacttttcatattatatttttcgtggatataacgtgattttataatagacatattcattatatttaggaatttaagcaaaagtaaaaaatttaaagtaacattataaaaaacgctaagggcctttggtaccaggcaattggatcatgagcactgcattaatataaatcatgagcacctcgttgttaaatcaggcaattcgattgtacttctaacgcgctttagcatttttaacttcacgcaatacatgagcgtgaaacatgtatatagcacgttaaaaaagaagaaagtctcgcatctactcggcggatcaatggaatatggagatgtctatcaatcgatatcaatgcgaggactaggaattgtcatgcaacggatgcacaaagagctataagtgtatgaaaactcaacaaaaactaagtaggtatgcatccaacttgcttcctcacgaagacctccggcatttgagaatgcccgtcatcggaatatacaattcgagttatataacgaaaaagtcccagtagtatatgagtgtgacaacataggagactctttatatgaagaacatgttgctactctgaagcacaagtgtaaaaaaagtatagtaacattgcctcttctctatttatctgttattttatttttattattttgttgggttctttttggccttttttttccatccggagtctcatcccggcttgtgggggaatcatagtctccatcatcctttcctcactggcacaatgttctaataatgatgatcatcacacttttatttacttacaacttgataactgaaacaatatgaccctataagaatgcctctggcagtggggacgagcgatggtcttttcctaccaatctatccccctaggagcatgcgcatagtactttgtttcgataactaatagatttttgcaataagtatgtgagttctttatgactaattattgagtccatggattatacgcaccctcacccttccatcattgctagcctcttcggtaccgtgcattgccctttctcacctcgagagttggtgcaaacttcgtcggtgcatccaaaccccgtgatacgatacgctctatcacacataagcctccttatatcttcctcaaaacagccaccatacctacctattatggcatttccatagccattccgagatatattgccatgcaacttccatcatcatcatatacatgacttgagcattcattgtcatattgctttgcatgatcgtaagatagctagcatgatattttcatggcttgtccgttttttatgtcattgctacgctagatcattgcacatcctggtacactgccagaggcattcatatagagtcatgtccttgttcagatatcgagttgtaatattgagttgtaagtaaataaaagtgtgatgatcatcattattagagcattgccccagtgaggaaaggatgatggagactatgattcccccacaagtcgggatgagactccagactttataaaaaaataaaagacgccaaagaagccgaaataaaaaaagaggccaaataagcccaccaaaaaaattaaaaataaaagaaaaaaagaaaagagaaaaagagagaaggggcaatgttactatccttttaccacacttgtgcttcagagtaccaccatgttcttcatatagagagtctcttgagttatcactttcatatactagtgggaatttcattatagaacttggcttgtatattccgatgatgggcttcctcaaatgtccgaggtcttcatgagcaagcaagttggatgcacacccacttagttttcagtttgagctttcatacacttatagctctagtgcatctgttgcacggcaatccctactcactcacattgatatctattgatgggcatctccatcgcccgttgatatgcctagttgatgtgagactatcttctccttttttgtcttctccacaaccaacattctattccatctatagtgctatgtccatggctcacgctcatgtattgcgtgaaagttgaaaatgtttgagaacgtcagaagtatgaaacaattgcttggcttgtcatcggggttgtgcatgatttgaatattttgtgtggtgaagatggagcatagccagactatatgattttgaagggataactttcttcggccttgttattttgaaaagacatgattgctttattagtaggcttgaagtattattgtttttatgtcaaatgatagactattgctttgaatcactcgtatcttaatattcatgccatgattagatacatgatcaagaatatgctaggtagcattccacatcaaaaattatcttttttatcatttacctactcgaggacgagcaggaattaagcttggggatgctgatacgtctccgtcgtatctataatttttgattgttccatgccaatattctacaactttcatatatttttggcaactttttatactatttttggggactaacatattgatccagtgcccagtgccagttcctgtttgttgcatgtttttgtttcgcagaatatccatatcaaacggagtccaaacgggataaaaacggacggagattatttttggaatattcggagaatatgggaaggaaaatccatgcgagacggtgcccgagggaggcacgaggcagcagggcgcgcccctgaccctcgtgcccccccccccccccggtaaggcggttgatgcccttcttcggccgcaagaaagctattttttggaaaaaaatcacgtcgcagatttcagtccaatcggagttacggatctccatatatatacggaacggtgaaagggcagcaaaacagaacgcagaaacagagagacagatccaatctcagaggggctctcgcccctcccatgccatggaggccaaggaccagaggggaaaccgttctcccatctagggaggaggtcaaggaagaagaagaaggggccccctctccccttctcttccggtggtgccggaacgctgccgtggccaccatcatcatcaccgcaatcttcaccaacaacttcaccgccatcatcaccaactcttgccccctctatgtagcggtgtaacctctctcttacccgctgtaatctctacttaaacatggtgctccacgctatatattatttctcaatgatgtatggctatcctatgatgtttgagtagatccgttttgtcctatgggttaattgatgatcgtgattggtttgagttgcatgtattattattggtgctttcctatggtgctctccgtgtcacacaagcgtgagggatccccgctgtagggtgttgcaatacgttcatgattcgcttatagtgggttgcgtgagttactgaaacacaaacccgagtaagggggttgttgcgtatgggataaagtggacttgatgctttaatgctatggttgggttttaccttaatgatctttagtagttgcggatgcttgctagagttccaatcataagtgcatatgatccaagtagagaaagtatgttagcttatgcctctccctcaaataaatttgcaataatgattaccggtctagttatcgattgtctagggacaaataactttctcgtaacaaaaagctctctactaaaactaatttagttgtgtctttatctaaacaacccctactttttatttacgcgctctttattttcttgcaaaactttccaacaacacctacaaagtacttctagtttcatacttgttctaggtaaagcgaacgttaagcgcgcgtagagttgtatcggtggtcgatagaacacgagggaatatttgttctacctttagctcctcgttgggttcgacactcttacttatcgaaagaggctacaattgatcccctatacttgtgggttatcaagggtcaggaacattgattggcaccttgaaagatttctcataattgaccctaagcccagtaaaagcagtataatgcacgatgaggtttttgacttgagcaagttgtctggcatcagtaggcagtactaggattgtatcatcaccatattggatcacaggaaaatctgggcaagcgtgacttctaatgggagaatgaattaaattctggtggatagcttcattgagcattgactgaagaagatcagctgccagcacaaagagtaaaggagaaacaggatccccttgcctgactccttgtctgcagtgaaaaagtttccctggcactccattgagcagaaccgaagaagtacctgaggaaagcaagattgtgatccagttaatccatctacttccaaaacctttggctttcagaatagcaagaatggcttgatggttaagcagatcaaaagctttctcaaagtctagtttgaggagtacaataggctgtttagattgttgacattgatgcagatattcaaaagcccatcccagacaatcatgaatagttctactcttgatgaagccatattgattagtgtgcacaatcttgagaatcacagtctgtaatctattggccaaaagtttggtaatgatcttgatagtgaagtttagaagagaaattggtctgaagccactggctgtcactggattgtccttctttggaatcaaagtgataaaagaggcattgatactctgaagggagatcttcccatgatagaaatcctcaatccacttgtagaaatcttgggtaatgatattccaacaggccttaataaaatctccattaaaaccatctgtcccaggtgctttgtcagaaggcaggtgcttaataactgagtcaatttcttgcttggtgaagggggcatccagttcctgcaagtcctcaaccctggtgatgaggttgattaggtttagagggtctgagatctctccagtctggcccagtctttctttaaatgcaacccaaagaattgcagctttttcatgatggtctgacatttctactccttgatcattgcataaactttgaatgtagttatgtctgtatttgatggttgccttagcctaatttttttagagttttcatcatcaaatttaacccatcaaattgttgctctttgtctccaataaatcctttgaaaagacagcaattttaacaaatgctcttttagcatttccttgccattttgttctatatctgtgagcactctgtattcctcaaaaagatcccacatcaggatgacattatttgtggcctgaatgttgctagctaggttggagaggcttttactccaaaattttagacctttcctgagtcttttgaattttccagtgatgagtttagcactgtcacttgccaaaatgggctgttgccaaatagattggacaacatcttgaaaatcatgattctgaagccagaaattttcaaatctgaagacttgagctctaggaatgcttgtaccaatttttatgacaaaaggacagtgatcagaaacaggtttggccaaaggaatagccatagtattgggatagttggaagaccaattttcagagatgaatacccagtcaattttctccagcaggggagcttgttgcatattgctccaagtaaaacttctacctttcaaaggaatctcaactagggccagttgactaattgcagcattgaaatccatcatgttattaatgtcaccattgcctacattcctgttagagggatatctgatataattgaaatctcctgtgatgatccaatcagattcaacaggcatctgaatgtttctgaaccattccagaaaattgtgttagtagaaaccaaggatgcatgctgatgcaccgtccagccaaaccgaaccaaactatgccggagtccagccaaaccgaaccatgccggataccaatccacgtaacgcaatttggatagttttgcaattcagtttgctatgcgtcgcacgtgaaggacggtctccggtttggatacgtccgacccgggttgtatccgatattttttccgcacgcagcatggtggcatgcatgcatccatggtgcatcggccccgccttcgagggaggtgctcacgcgtggctcgctggccccgcctcgtttgccactaccatcatgcacggcttgccggactggcctcaatttgccgctgccgtcgagcgccgctcaggcgcagctctctggacctgcctccatagccgccatcgtcgcgcgcggcttgtcagaccgggaccgtcctccatagcagctaccgtcaagcgcccctcacgtgcggctccctgccctgcctttgcggtctctgtcgttgcgccgcttgtcagactggccttcgcgcctccatgaccgcccgtggcacatgacatagtgcgaaggtatgcatgtgcaaatgagtaacgcatcacaaattttgttcattctaaatgatcaagttcatgggcgccattatcttcttgaagacgtcgtggtgctcctcttcgtgcctaggttccgagtgaaaacctttgtccgttttggactcggcagcgatgacgtgttgtgccgttctccctccctaggacgttgttgtggagcttattaggtgttattggtcgtagcgtggtgttgtaaacagttcctcccgtgctctgtcttggtagcttagtcgcgtgagtcttgtgtggtccgattgtcttgggatcggtgttgtctgggattacctcatcaccctgtatcgtttagtcgtgtactttgtttgatctttgctttatatatataaagcggggcgaaagcctgtttcaggatccttcagtgacgttctccttcccgagggcgttgtcttggagcaggtgctggctggagggggcatgaggtggtgcggtgtgtcatctaccacgttggtgacggcgagtgtcggcagcatggcgcagtgaggtcccggagttggaagtgtgttgatggacgcgcatatgatggtagcactgtctagcgtcatggtggcatcgataacagttgggccctggcaaggcctatccattgatctctcctgaaaatgggatggtggaagatggcggtggcagactcgagagagtgcgcatgcggtgcacgctgaaggtctgctagaccggttggtgttctcagctcgccgtggggcaacctggtgaggccaccggattagatggcgtgcgtggatgcgccagtgcactccatcagacttgtacgtatagcgtttaggttgccaggaaggatgctttgggtccatccatctatctgctttgtcagactttgtttaataatttttaaatatggttgcatgcatcattttgatgcagaggcaggggtaatcctccttttcgaaaaaaaaccaggcaagaaatccgtttctacatgtaaaattccctttgctaaaatatgtaaatttccgtcttaaaaatggaatacatcctaacggaattctttctcaatatctgcaactataaaccacctaaagaaatccctgtcaaaaaacatcgcccaaggcaaatatctcgatggttcttgattttgctgtgttcacttcattgttactcaacactaacgtgcctggcctagcacgagaaagagaggttggaatcatagcccctgcctttaagggcagaagaaaaagattatttgaccaagggttctcagttctcattcatggaaacttcgtgcgggtcccagggagacctgccaagtccaagtcttccccatataagaccgtgacatttttgtttttaagaggcggaaaaagccatggacctgtatactagtcttttctgaggctagtgtttgtgagaacgaccatgctcgatgtggaagtagtttggtcaactttgcttcactaccaccttctttacaagtactcccttcattcctaaatataaaaccttttagagattctactttgaactacatacccatgtatgttgtccataatgaaatctctaaaaggtcttgtatttaggaacggaggaagtataaaacataccccaaaaatctcaactcacaaacatttcaagccaatcaaacaatttggatagctctgcctgtagtaaagtggagtactttgtttaaagaaatataacatatcctcaaaataactggactcaatatcatttccatccagtaaaataagttggatatatagctgtgcatctattgatgtggatggctgcaaaagctatctacaccactcaaacagacgttagccggctaatgttgctttcaacagggattggaccaaatccatacaaaaatcacccgaccttacgggtcaaaaagttgaaaaaaacttctcgcatgtagctaccagaatgtctcgtgtgcattcgcagagattcatatgaaatgacttaatttatgattatttttcgctacttctgcacacatgtctcaaaaacataaatagttgtgccaaatttgaaacttcacataacatattttggattcataaaagattttcagttcactcaacatattttcaatgaaggtgttgacgttaatcagtggtatagagcatagacgtgtactgctcgtctacagctatgtagcagaagtacacccattgaattagctaactctagcgacaactcaatccatcccgtcacaacccagaccgcgcgcggggcgacgaatggtatgaggcccaagcgggacgggtcagccacgtgggagactatgggtagaatcggagaacgggccaaatccaaaaaaaaacagcccacctcatgtgctcacttgaatttataaaattaaatcaaatttgggttttgaagcgtcaaaaagttcaaaaacaattctcgcatgtagctaccagaatgtctcgtgtgcatttgaagagatccataagacatgacttaatttatgaataagtttccccccgcggtttgcttaccaccttctttatactacaagtataagacatacaccaaaatatctcgactcgctaacatttccagccaatcaaataatttggtagctctacctataataaaatggagtagttcaaaaaaacttgtccccaaaatatgaggactcaatcccatttcgaaccaatcaaatatatatagctgtgcatctattaatgtggagggccacaagagctatctaaaccactcaaacaaacgctagctggctaatgttgctttcaatagggattggacgaaatccaaacagaaaacagcccaccacatgtgctttctaaaaaatttgtaatttgggttttgaagcgtcaaaaagctcaaaaaccaatctcgcatgtagctaccagaatgtctcgtgtgcatttgcagagatccataagacacgacttaatttatgaataggttttgttatagtttcacagatgtctcataaacataaatattcacaccaaagttgaaacttcacataacatgttttccatttttaagagatcttcagttcgcctaacaaattttcaatgacagcgatggtctcatgcgtgttgacgttagtgagtggtggtatagagtatagacgtgtaccactcgtctactcctatatgtagcagaattgcgccaactgaaattagctaactttagcgacaggtcaatctatctccgttccgccgtgatgctaacgagccggtgcgtattcatcacagcggtgctgcaactactaatctccttcctggcggtcgccggggaaccacaaatcgggctgcccggctgccagacccgctgcggcgacgtgagcgtgtcgtacccgttcggcatgggacccaagaagtgctactggccgggtttgaagctcacctgcgacgaccgcggaagcaaacccccgcccagtatttcgccgcagactacaactccgacagctgctccaacttgggctgctgccagtcgtccatcttgtccagcagcacgtcctatgatgtcgaggtcaatcggctcggcgattgcctgcggtacggccctgtgcccgacccgtttcccgacgatgttccggtgaatgtgctcatcgctgagaagggttggttctaccaggagtggtcacgcaatgtcataaatgttacctcgcggcccaccgtgattttcgagtggcgggtgccgcttggtgccccggtcccggtggggccgtgccccgacgacgcagcccggagcatctgcaagagcacccatagctattgcacacaagagtggtcaaataatacagtcggggcctattcttgccagtgcaactccggctacaccggcaacccttacctcaccgatggatgccaaggtgagttcacaacttcacatgtgcacatgtccatgttttgttaacttaattacagtatcttttatttacttagtcttaaacaagacatgctaaactatattgtgtgcagatatccatgtgtgtgatcagaaagaaaaacatggctgcttcggccattgtgagcgactgcccggatatgttagctgccggtgcccagaaggaacccatggcaactactccatacccgggggctgtgtcgcagacacaaacacaggtatgacacgcaccagccagtcgattactactactagtacgtgcaaacaatggaactgttattttaatgggcctgcttaagcaattagttatagtaaacatatgtgcgtgtattgtttaactttcaggtaacttggccttaatcattggtttgtcggctgcaagtggcccattcattctacttttggttcttcgcatactcgtattgtcaagtgactttaaggaacaaaagctgaggatgttgagacggaagttctttactcaaaaccgtggacaactgctgaagcagttggtatctcatagggcagacatcgcagagaggatgctcatttcgttagaagagctacagaaggctaccaacaatttcaatcaagctcgcaggcttggtggtggagggcatggcactgtctacaaagggatcttatcagacttgcatgttgtggctataaagaagtcaaatattgttgtgaaaagagaaattgacgagttcatcaatgaagttgcgatactctcgcagatcaaccataggaatattgtaaagcttcgtgggtgttgcctcgagacagaagtccctttattggcatacgagttcatttccaatggaacacttagtgatcatcttcacacggaagaaccaagatcgttaacttggaaagataagttaaggatcacaaccgaaacatgcaaagctcttgcataccttcactctgctgtttcagtccctgtaatacatagagatatcaagccttccaacatacttcttgatgatgccttgacagcaaaagtgtcagactttggagcttcaaggtacattgccatgaatcaaacaggaacaacaactgcagtgcaaggaactataggttacttggatcctacatattattatagcagacgcctcacagaaagtagcgatgtttatagctttggagttcttcttattgaattgcttactaggaggaagccatctttgtatagatccaatgaaggcgttgggcttgtcatggagttcgttgcactacttgcagaaggcaatctatccgaaatactagacccaccagttgtagaagagggaggtagcaaagtcgaagacgtagctaatctagctgtgtcgtgcgtgaaactgagagcagaggagcgaccaactatgaggcaagtggagatggcgctggaagctctccaagcacgcaaggagcatgtcatgggtgatttgatagaagaaacaaacgggaagaaacatgcagcaccaaattgtccatcgactagcaaacgaccaaagggaagtggagcaagcagatgctatagccaagaagaagaggtggtgttatccgcaacattccctcgatagttttgcttgcccggaagtgatttttagtgatgttgtattctttctactatttggaatgagcgtgtgctattgtatgaatatatgagttacacataactctagtgtattatttaaaataaatttgaatgcacccaactctgttgtgctaattttgcatgttgtcgcgcaatcagcatttggtcttgatgatcgacagttcatcactagtggaaaaagtgttagtcacaatttttgttggtggcgcaccgactcctaacaacggtagtactattttttccaaataatggtggcgtcggacaatttggtacgacattgatttgagcataccgctggcatagaatttttctcgtaccacataggcattttctgagtttttttccgtgtgctttcgttttctatagcgtggcccattaggcatacgacagcggtatccattaggcccacgcgagcaaaataaaactaccctatccagtaaagatcagtgtaggtccgattcactaacctatcattttcgcctcttcttcatcccccttctcgaccgccccgccaccgccactgcccgatgacgccgctcttcgccgccggaactgcgcggccgccgccaactccggcaaggtgctacactgtgtcatgtttggtcgataggtgctacgcacgacaaatcctttgcgtctggatggacgagcgcaggacgatagcgtcgtcgggcgtcgtggtggcatcgacggaccggtaaggatgatgcggatctatctcctgaagatgggtcagcggtccgatgatgatggcggcttctaaaacgtgtgcatgtgttgtacgcattttgtctgctgcgccggtgttagttctgatacattatgtggatggatcggcgacgacactggttttagatatgggagtgagagccctccacattatcgagttttttagatgtgagtagtggtttcgggtggcttgatgtatattcctgttcgacctttgttgaataataaataaagatgaccgtatgcatcgattgatgcagaggccggtgttttaacctcctttttgaaaggaaaagtactatgttagtagagtgcttagctgattaaggatgaaaactgcaatagctccttactttccctggtaaaactacaaatatcacaaatgcaaacccacccatcccggtagcctcgtcaaattaaaataaaaaaaaatataagaaaaggaaaatgcgaccggcggctagcagctccacctaccgcagctggccggtcgtcggtccttgcatcgcatccaaggcgacgccggctccaccactgccgccaccactgattggtaccttaagctcccgtgaagctacaagggaggaggccccctcgcctcccatccattgttcctcaacagcttgggtgccgagctcccccaccaccacactagacgcgctgggattcattggatccgctccagcgagcgagccggattcagttcaccgagattatattcacccttcccgtctgccaactgattacctcccttttcccattctaccctgggtgaccactctgctcactctcactctttctttctcctctacgccggccgtgcacagcgcgacgccgacgaccgcatccccccgacgttgccgcagccgccatacaagtagaaggtgaggacccccttcctctcctcttcgtcctagccagcggatcctcagatctgagctgagtggggccgcagcaagctcagactaaattgtttcttacaaatctttgagatgatttccgtaccacgtatagaactcctaatttctcagcagaagaaatcaccgggttctgggtttgcgcacaaagctttgattttgttttgtgctgtgctgtgaaaattgagctcagatcttcttttagtagcctgtgatttgtgcagtccaatttgctgtgcggtaccaactaagctcacatctttttagtagaaagtacctagtagtttttagagctttgctttgcaagtagtacactagtactacaaattaagctcacacattatattattacagaggctctgttttgttcagtactacaaagcttagattttgatttctgtactacgaatttagctcagatcttttttctgaacagcaagcttttaatttctgcaaataggaccgagatggcaacctctcccagctttgtgctacaccgcaagtactaggagcattgctgaatgccggatatagatccccagatctaggccaagggtctcgctttctgctcactgttacttctatcatctctccaatcgatccaaggtaattcatcgattgcagcagcaccaccctctatttagtgtgcactttcttttgtgtgcaatccatgcttttcctttacaacgaattgttggtagtctctgctgagtgaatctacatgaccatccttcttttccattttttttgcatgtcactattgatgtgtgaaaggtagtaataaagaggactcattttgtgtgcatcctttgttttcagttccagctcaagccactggaccctgcaactacttgcgagacagcacgggatatctatctctgcaacaagatccgtctctcatctctctagtcgattcaaggtacatagctgaatccagctacacaacacttactctagttatttttcttttttgaaagagctgatcgtgtgtctttccatttcaattgttggtgtttgttcaaggtaatactatatcggttttatttcgagccgaatttctgtgcactgtctttgcaagccacattttcctttggatttgttactagcctctagtgagtgaatctgattatccttcctgttagcatgggattgttgatgtgaaaaagcgaggtagtaatacaaaggactaatttttatttccatgcttcttttcagtactagttcaagcgtgagcaaaccctgcaaccaatggcgggggttctggatgctttggcatcctacgtgaccaacatgctcaccgagatggctaaagaggaggtggccatgctaatcggcgtgtctgacgggatcaaagacctaagcatcaagcttggggacctcaagaatttccttgctgatgctgataggaggaacattaccgatgatagtgtgcgggggtgggtgggcgaactgaagcgtgccatgtacttggccactgacatcgtcgacctatgtcagctcaaggccatggagcaaggtcaaacaaaggacagggcgtgccggtgccttaaccctctgctcttttgcatgcggaatcccctccacgcccacgacatcggcacccgcatcaagctgctcaaccaaaatttggatgatatttgcaagaggggcagcagtttcaatttcatcaagctagaagcctaccaagaccaaaagaccactcggtctcccgccactgaccggaaaacaaattcactgattgagcggtccggtgtggttggagagaagatcgaggaggacacgagggcacttgtggaggtgcttacaagggaggcggtaggtgacaagagtggtcgcctcattgtggtcgccattgttggtatcggagggattggtaagactaccctcggcaagaaggtcttcaatgatgaggccatcgaaggcaagtttactaagaagatatggcttagcatcacacaagatttcaccgatgttgagttgttaagtacgaccatcactgccattggggcagatcttcctggagggggtggggctccagacaaggccctacttgtcgatgctctcaagaacgccatcaaggacaagaagttctttcttgtactagatgacctgtgggatgtcgatgcatggaacaaacatctaatgactccctttagctatggtggccccggtagtagagtcctcatcaccaccagacatgacactgtagcccgaagcatgaaagcctttcatccctaccatcatgttgacaaattagctccacaagatgcttggtcgttgctcaagaagcaggtcggtacttcccaaaactcaatataatacacgtcgtttgggactacactgttaagttaatttgatctacacttgcataagtctaccaatctgaaatttatatatttataatgcttccttgacttaaatttcaccgtaacacgagttcatcaagtttgtatatgaaattaggaagatattaaacaatattttcatttgtatgcatgatgtacggcttctcaatttgtggattattccggacttaagtttagcaattatcagggattgcatccagcttctcaattagtttctacttgcaggtagtcacaggagaggaaaatgaaccagaagttgatatgctagaagatattgggctgcagattatagcaaaatgtgatggcttaccacttgctgtaaaagttatgggtggactcctatgcaagaaggagaaaacacgacgtgattggcaagacgtcttgaatgatgatatgtggtcagtatctcaaatgtcaaaggaactaaattatgccatatatcttagctatgaggatttgtccccttacttaaaacagtgcttcttgcacttctccctcaaaccaaaaaagacagtgataactgatactgaaatggtgtccatgtgggttggtgaaggattggttgaaggagacacatatactcgtagtttggaagaagggaataagtactataaggagctaatagtaaggaaccttatagaggtagatacaaagtaccctagtcaacttatttgcaacatgcatgatgttattcgctcatttgctcaatttgtggctagggatgaaacactagtaggtcacaatggagatactatcaaaacaaatcttagatcaccgaattatcttagattatccatagaaacgaaaggagtgggatccgatgaatttgagtggagatatttaagagagcaaaaattgcttaggtctctaatattaactggaaacctcaaaagtcagcctggggattcgttgactatcttcccaagtctacgtcttttgcatatagaatcagcaaatattgctgcactagttgaatctatgtaccaactcaagcatttgagatatttggcattaaagaggactgatatgtgtagactaccagagaacatccatgagatgaaattcctacagcatattagccttgaaggttgtgaaagtttcatgaaacttcctgatagtattatcaagctgcaagggttgagatatcttgatatgggtgacacacgtgtaagtagtattcctaggggtttccgagctcttacaaatttgacttcactatttgggtttccagcctatattgatggtgactggtgtagtctggaagagttggggtctctttcccagctcaatgaactttcactacagagcctagaaaatgtatctagtgccttgttggctgaaaaggcaagggtaaatgcaaagaaacaacttaccgtacttgctttaaaatgtggtggtagagtgggacatgggttggtccaaggagaggtctctgagtctaaggaggaggagcaaataattgaggcggtgtttgatgtgctctgtcctcagccttgcatagaacacatcagaatagaaagatattttggtcgtcggctcccaggatggatggcgtccacagctatggtgcccctcgagagcttgaagattctatgcctcgaacacctgccctgctgcacccaactcccagatggcttgtgcaggctcccgtatttggagtggataaaagtgatgaatgctccagtaatcaagtgtattggtcctgaattcgttcaacagtacaatcagctgcaccgtccttcatctcagttggctgctacgtttcccaaactccagatgttggaatttcacggaatggaggaatgggaggagtgggtttgggagacggaagtgaaagctatgcccttattggaggaacttcgtatcacttcttgcagactgagccgtatgcctccaggacttatgtctcatgcaatggctttgaagaagctaacaatatggagcgtccaatgtctccactctctagagaactttgtttctgtagttgaactcgaattgggaaacatacctgaactggccatgatctccaatcttccaaaattacaaaaacttacaatcgagtgctgcccaaagctcgagatgctgcaggagatggctgcactccggagactcgagctgaccattttcaacagcgaaaatcaacttccggtctacctgcagactgtgaagcctagtaatttgctgctgacctgcaacctagcggtactcacttccatggctgagggtgaatctagctccgagtgggacaagttcagtcatatcaaccacgttgaggcttatgcagaggatggagaagatgagaagaaatggcacgtgttctacacatctgaatcctgcaacatagagacaaatattcatcaggtaatactttggtctctccctctttcaatctagctaataataatattcttccttattgttgtctgttccatgcatatctattttcatcagtatgatataggatagctgaatatatctcccactgtttttgttttgcttgccaggatcgattggtcgaagaagaggagtaggctgaaactccagccgaacgaggaaggaccatatgatgcaaggatatataagtatgtctgctgttacaacttcaactagttttgagatcgaatccatgaagggatacggggaaaagcatcagccataatgccatatacacttacctgcagagattcacacatcatactaatttcttgtgaagtgtgacatatacagttacgaatttagagatgtaaacttcgtggcggactatccagctggtgaagaaacatggtgaccttggcaaggctctcctttgtttagtgcaagcaactaatggagtttagactactctgctttgctctgctctctgaaagcagctcaggttgcaggtcctctgaagcagctgcgtttttctttttcttttttcgcgggtgtctttcattcgttctctggaaaactatgtttatttctgatagatcaatcaatagtatactggaacactaaatactgttagaacaaacccaatcaaaatgtactaatgctctgcacctgtgagccaatcaaacggatgtatatcaaagagaggcatcatattattgaggagccatcggagattttctgaatttgcccagcttgaggatggatctgggccgccgccgccgccagcgttggggccgcagctctgtacgcgatttgggattgaacgatgaggccatcgagaccaaattagcttgcagggaaggacctttttgcaaattatgcgcctaaatctgggccatcattttcctatccggtggtccagatccactttttcgatttttctaccataagcatgttttctgttgtagttgctcctcaacagttgtacgtattttgatggtagatggatcatggatggatgcataaggctggtcatagtgggaagtatcatatactagtatcatgcatatgatactagtgtataaactacatccatagtgcatagtatcatagattagtatcataggtggtctcatttattgccatgcatgacacatagtagcattacattaattatgttacggtatctacctatgttactataactatctctctcttctttaattgcctgccacataagcatgtttgcgattcccaagtgcatgatactacttatgttacttccactatgaccagcctaatgcatcttcacaatcatttggcatcactggccgccggccaccgtttttactccattattttttgttcagtgggtagtaaggaaccagtaacaattaataactggttaatagatgcatggatctgataaataagccaactatttagcaactttaggtgctaacttattaaataaggtgtgcttagcaataacaggttaagcacctatacattgaggagttgagttgctaagatatttaatgcacttaacatctcatttaagcacctttgcatttgaagaggtcaaagtgacagctagcttactcagcttaagataatttgagttccggaaaaggttttcgtcccgctttatataattcaatcgaccgttcacatgcaggactagctgtacaacacagttgatgctacttgctatagtgccacatgggtatctgtaaccattccgtaattaatggtttaacccaacggatggagcttgacccgttagacttgccgctaagactacccacaatgagagtaacataggtagtaacatcacacatatctagataaaatagataatgtggcaagcaataaatgaagaaagagaggcatgtagtaacatagctagttagtactactagtataagtaacatcacacatagctacttagtactagcataataaatgaagtgtcacagatgttactccccactatagaggtagtaacatagagtagtaacatgggcatgttactactctatattactacccattgtggctagtctaagcgtgcgagtcgtcgtcaaattttaactaatgtgctacaacttccattggaggaacttcagatctgttcttgcaaactgggttatttgcctctaggacttatgtctcatgcaatggctttgaagacgctagaaatatggaacgtccatgctctcaactccctagagaactttgtttctgtagttgagcttgacttgttagacatacccgaattggtcaagatctcctatcttccaaaattacaaaagcctaaaatcaggtactgcccagagctcaagacgctgcaggagatgtctgcactccggagactcgagctgaccattttcaacagcgaaaatcaacttccggtctacctgcagactgtaaagcctagtcatttgctgctgacctgcaacctagcagtacttacttccatggctgacggtgaatctagctcggagtgggacaagttcagtcatatcaagcacgtcgaggcttatgcaaagggtggagaagatgagaagaaatggcacgtgttctacacatctgaatcctgcaacatactttggtttccctctctttcaatctactagctaataatattcttccttaatgtaatctttgttggttccatgcatattgttatcatcagtattatataggatagctgaatgtatctcccactattttgttttgcttgccaggatcgattggtggaagaagaggactagaccgaaactcctacggaacgagtttaggcgaaaggaccatatgatgcaaggatatacgtatgtctactgttatagcttctactagttttgggtattcttacctagtgccatgaccattggaatctcatgtttaatattatgatcgaatccatgcagggatacctggaaagcatcagccataatgccatatacacttaacctgcagagattcggacaccacactaatttcttgcgaagtgtgacatatacacttactaattttgagatgtaaacttcttggcgtactatctagctggtgaagaaacatggtgaccttggcaaggctgtcctttgtgcagtgcaagcaactaatggagtttatgctactctgctctgctctgctctgttctctgaaagcagctcaggttgcagcttctccattgtggcgtttttctttttctttttcacgggtgttttgcgttggttctctgaaaaactatgttttttttgatagaccagtcaatagtgtactggtatttcagcttttaatttgtactgcaaccacacaaatgactgtcagagagtgtagtttattcaagcttccggctgctgatttgtaactgtatgtcataggaattccgaatcagagtgatgtatactgggaccaaacaaatgttggtgagatcctggtccacgaagatcacgatgatgacctgctgactggatgttctagctatctttagtttcttcaattagtgaaatcaaattagatcctggctaatatggtcaaatccgtggcacgtgggtccacgaagaacacgtgggtctagctatctgttgtttcttcaatcagtgcagtcaaattaagttcaggttttccccgcaaaaaaaaaaatttaagttcaggtttgttctggggctcaggacatatgttgtggatggaagcaactgtatcaggacatattggatcaggacatgaaactgtaattgcaggcatcaatgtatgtacctgcgcgtcttttctttttatgaatgtgtgtacctgcgcgtcaatgcggacgatgcagatcttgccgtccctcgtgcgtcctcgaagggcgcatcatctaaatgagaagcaggcttggtgcagccgtgctgagatcctctcaagggaaggtggaagggagggcctggagcacgacatcctccttgcggacttacctggcgccggtgctcctgtactgcagtggcgtacgggtttgatgatctgctcctttctatggagaagaatgggtgtgctgccaactcccgtatgctaaatacttgtatagttagaaggttacttcagaaagggggaatgcccagggctgggatttgtctgtctaaaattgatgagaggatcttcacccttgaagcttccacacctagcttgttttttttcttttttgcatgggacacctagcttctaaaatttaatcaagcaataagtagtatgtgaaaatgaaggaaggcgaatcaagctgtatgtataggtacgtgcagaaggtaggtgagtgaaggacgagatttccaatggctgcaaaccgtactgcatatttcatgcacccacggccaggtttgatcgttcacatctctacatggccattataaatttacactagtccttgatgctagcttgcagctttcttggccttcctaggcagctatactctagaggttgtggttgccacttcactacatgattaaatttctccatggataccatctatgtatgtgtgcgcgtcgttgatacatagttaggtggtgggattgtgaggcagcagaaatctgattgagcagtaaaataaaggtatttgcactatgatacagcgacagcgaaaaaagaatagtgcttgcagtgttgcggaggagctagatgtgtcatcccaatagtgggagaagggttaaggagggtatcgagctagggagagatggtgggtctgtgtggtgggtgtgtgaaccgctgcagccttagtgaggagcgtgtggttacaagggaccatctagcttttttccgtttggatgagtgcacgtggttacagaagccctagcattagtggggagacagccaggcctaggacacagcagaattatgtgatttagcagcacaaaccaagtgtctgttggcatgcttgttcgaaggccaaggttcaatcactatggaatttt

SEQ ID NO: 11 - DNA, 22 bp, Artificial sequence
  Primer
tgtgtcatgtttggtcgatagg

SEQ ID NO: 12 - DNA, 20 bp, Artificial sequence
  Primer
tcctcccttgtagcttcacg

SEQ ID NO: 13 - DNA, 24 bp, Artificial sequence
  Primer
gcttccttgacttaaatttcaccg

SEQ ID NO: 14 - DNA, 22 bp, Artificial sequence
  Primer
ccacatatcatcattcaagacg

SEQ ID NO: 15 - DNA, 22 bp, Artificial sequence
  Primer
agatgagaagaaatggcacgtg

SEQ ID NO: 16 - DNA, 23 bp, Artificial sequence
  Primer
ccagtatacatcactctgattcg

SEQ ID NO: 17 - DNA, 20 bp, Artificial sequence
  Primer
atattcacccttcccgtctg

SEQ ID NO: 18 - DNA, 20 bp, Artificial sequence
  Primer
cttgccaatcacgtcgtgtt

SEQ ID NO: 19 - DNA, 20 bp, Artificial sequence
  Primer
gcaccgtccttcatctcagt

SEQ ID NO: 20 - DNA, 20 bp, Artificial sequence
  Primer
tgcttttccccgtatccctt

SEQ ID NO: 21 - DNA, 21 bp, Artificial sequence
  Primer
tagttcaagcgtgagcaaacc

SEQ ID NO: 22 - DNA, 20 bp, Artificial sequence
  Primer
ccatgtttcttcaccagctg

SEQ ID NO: 23 - DNA, 22 bp, Artificial sequence
  Primer
ctgtagttgaactcgaattggg

SEQ ID NO: 24 - DNA, 20 bp, Artificial sequence
  Primer
atggctgatgcttttccccg

SEQ ID NO: 25 - DNA, 20 bp, Artificial sequence
  Primer
actacttgcgagacagcacg

SEQ ID NO: 26 - DNA, 22 bp, Artificial sequence
  Primer
gaagcatgaaagcctttcatcc

SEQ ID NO: 27 - DNA, 21 bp, Artificial sequence
  Primer
tccattagttgcttgcactgc

SEQ ID NO: 28 - DNA, 20 bp, Artificial sequence
  Primer
tgagagacggatcttgttgc

SEQ ID NO: 29 - DNA, 20 bp, Artificial sequence
  Primer
agtagttgcagggtccagtg

SEQ ID NO: 30 - DNA, 20 bp, Artificial sequence
  Primer
aaagctcgagatgctgcagg

SEQ ID NO: 31 - DNA, 20 bp, Artificial sequence
  Primer
tccgagtgggacaagttcag

SEQ ID NO: 32 - DNA, 22 bp, Artificial sequence
  Primer
cacaggagaggaaaatgaacca

SEQ ID NO: 33 - DNA, 21 bp, Artificial sequence
  Primer
caagaaggagaaaacacgacg

SEQ ID NO: 34 - DNA, 20 bp, Artificial sequence
  Primer
tgtggctagggatgaaacac

SEQ ID NO: 35 - DNA, 20 bp, Artificial sequence
  Primer
catcatatggtccttcctcg

SEQ ID NO: 36 - DNA, 22 bp, Artificial sequence
  Primer
gcaaaatgtgatggcttaccac

SEQ ID NO: 37 - DNA, 20 bp, Artificial sequence
  Primer
actagtgtttcatccctagc

SEQ ID NO: 38 - DNA, 20 bp, Artificial sequence
  Primer
tgtgcactgtctttgcaagc

SEQ ID NO: 39 - DNA, 20 bp, Artificial sequence
  Primer
gtgtagtcccaaacgacgtg

SEQ ID NO: 40 - DNA, 20 bp, Artificial sequence
  Primer
gcatgatgtacggcttctca

SEQ ID NO: 41 - DNA, 20 bp, Artificial sequence
  Primer
gagtggagacattggacgct

SEQ ID NO: 42 - DNA, 20 bp, Artificial sequence
  Primer
gatgaagatagggatgccgg

SEQ ID NO: 43 - DNA, 20 bp, Artificial sequence
  Primer
agaacttctgtctcagcgcc

SEQ ID NO: 44 - DNA, 21 bp, Artificial sequence
  Primer
tagaacaacatagttgggtgc

SEQ ID NO: 45 - DNA, 20 bp, Artificial sequence
  Primer
gtgtcggagactttcaagtc

SEQ ID NO: 46 - DNA, 19 bp, Artificial sequence
  Primer
gatgtcggccctgtgagaa

SEQ ID NO: 47 - DNA, 20 bp, Artificial sequence
  Primer
tttctgcttcggggactgtg

SEQ ID NO: 48 - DNA, 22 bp, Artificial sequence
  Primer
aacagaaacaattcaccatggc

SEQ ID NO: 49 - DNA, 20 bp, Artificial sequence
  Primer
agcgagtgatatagatgcgc

SEQ ID NO: 50 - DNA, 20 bp, Artificial sequence
  Primer
tgcaaatggccagagttcac

SEQ ID NO: 51 - DNA, 20 bp, Artificial sequence
  Primer
cttcacatgtgcacatgtcc

SEQ ID NO: 52 - DNA, 23 bp, Artificial sequence
  Primer
tattcatacaatagcacacgctc

SEQ ID NO: 53 - DNA, 20 bp, Artificial sequence
  Primer
tctgcaagagcacccatagc

SEQ ID NO: 54 - DNA, 20 bp, Artificial sequence
  Primer
aaaatcacttccgggcaagc

SEQ ID NO: 55 - DNA, 21 bp, Artificial sequence
  Primer
gtcaaataatacagtcggggc

SEQ ID NO: 56 - DNA, 23 bp, Artificial sequence
  Primer
tgaaggtatgcaagagctttgca

SEQ ID NO: 57 - DNA, 20 bp, Artificial sequence
  Primer
acacaggtatgacacgcacc

SEQ ID NO: 58 - DNA, 20 bp, Artificial sequence
  Primer
caagcctgcgagcttgattg

SEQ ID NO: 59 - DNA, 20 bp, Artificial sequence
  Primer
tatgccagcggtcgaacaac

SEQ ID NO: 60 - DNA, 20 bp, Artificial sequence
  Primer
ggaacagcacctcagggcac

SEQ ID NO: 61 - DNA, 727 bp, Aegilops tauschii'PI511383'
tgtgtcatgtttggtcgataggtgctacgcacgacaaatcctttgcgtctggatggacgagcgcaggacgatagcgtcgtcgggcgtcgtggtggcatcgacggaccggtaaggatgatgcggatctatctcctgaagatgggtcagcggtccgatgatgatggcggcttctaaaacgtgtgcatgtgttgtacgcattttgtctgctgcgccggtgttagttctgatacattatgtggatggatcggcgacgacactggttttagatatgggagtgagagccctccacattatcgagttttttagatgtgagtagtggtttcgggtggcttgatgtatattcctgttcgacctttgttgaataataaataaagatgaccgtatgcatcgattgatgcagaggccggtgttttaacctcctttttgaaaggaaaagtactatgttagtagagtgcttagctgattaaggatgaaaactgcaatagctccttactttccctggtaaaactacaaatatcacaaatgcaaacccacccatcccggtagcctcgtcaaattaaaataaaaaaaaatataagaaaaggaaaatgcgaccggcggctagcagctccacctaccgcagctggccggtcgtcggtccttgcatcgcatccaaggcgacgccggctccaccactgccgccaccactgattggtaccttaagctcccgtgaagctacaagggagga

SEQ ID NO: 62 - DNA, 361 bp, Aegilops tauschii'PI511383'
gcttccttgacttaaatttcaccgtaacacgagttcatcaagtttgtatatgaaattaggaagatattaaacaatattttcatttgtatgcatgatgtacggcttctcaatttgtggattattccggacttaagtttagcaattatcagggattgcatccagcttctcaattagtttctacttgcaggtagtcacaggagaggaaaatgaaccagaagttgatatgctagaagatattgggctgcagattatagcaaaatgtgatggcttaccacttgctgtaaaagttatgggtggactcctatgcaagaaggagaaaacacgacgtgattggcaagacgtcttgaatgatgatatgtgg

SEQ ID NO: 63 - DNA, 858 bp, Aegilops tauschii'PI511383'
agatgagaagaaatggcacgtgttctacacatctgaatcctgcaacatactttggtttccctctctttcaatctactagctaataatattcttccttaatgtaatctttgttggttccatgcatattgttatcatcagtattatataggatagctgaatgtatctcccactattttgttttgcttgccaggatcgattggtggaagaagaggactagaccgaaactcctacggaacgagtttaggcgaaaggaccatatgatgcaaggatatacgtatgtctactgttatagcttctactagttttgggtattcttacctagtgccatgaccattggaatctcatgtttaatattatgatcgaatccatgcagggatacctggaaagcatcagccataatgccatatacacttaacctgcagagattcggacaccacactaatttcttgcgaagtgtgacatatacacttactaattttgagatgtaaacttcttggcgtactatctagctggtgaagaaacatggtgaccttggcaaggctgtcctttgtgcagtgcaagcaactaatggagtttatgctactctgctctgctctgctctgttctctgaaagcagctcaggttgcagcttctccattgtggcgtttttctttttctttttcacgggtgttttgcgttggttctctgaaaaactatgttttttttgatagaccagtcaatagtgtactggtatttcagcttttaatttgtactgcaaccacacaaatgactgtcagagagtgtagtttattcaagcttccggctgctgatttgtaactgtatgtcataggaattccgaatcagagtgatgtatactgg